European Patent Specification EP 3 641 833 B1, published July 23, 2025. Title: Methods and compositions for controlling cardiac fibrosis and remodeling. Applicant: Université de Lausanne. The sequence listing filed with the application follows.

SEQUENCE LISTING (14 sequences)

SEQ ID NO: 1 - DNA, 5359 bp, Homo sapiens
gtcccctaccccatgattcaaagcagaaattcgcaaagactttgatgtaggctgggctgggagttgactacacttgcatgcctgttgcttggcaggatggctttcaaaaaagaaaaaaatataataatgaaagattgaaaacagattattggggagaaaagtatcccaggcgctagacggctgtctctgcagcctctggctcctgtcccacccattccccggccctgacgcaaggctggctggaagaaggtgttctcgagattgttcaggctgagggcctgactggcaggagactgaagcctaccccattcctgcctgggtgccaagctctgcatgaggtttaaatatacccacagcctgacactatgccctagatcatgctaaatgtttccatactccttgaattctcttctcaaggttcatttattgtccccatttttcagatcagtaaactgaggcccagagaggttaactggtttgcccacagtcacacagccagacaagtttgagtatgtctgattctattgccttattccaggtttgggatacaggcagagtagggagaggtttaggatggtaaagaagaatgttccaggaggaacagagttagtgtaagggcagtctaatctagagtcagaatttggagctgtttgttacagcagcatgacctagcctatcctgactgatacaaatcatggtaaactaatttatatgtcctgaaaaatattagaacttagcatctacctcttaggagagcttttttttttttttttaacttttacattttggcaaaacacaccgaacataaaatttaccatctaagcaattttaaatgtacaatgcatggctttaagtacattcacattattgagtttctatcaccatccttccacagaactcgtcatcttgcaaaactgaaattctaaacccattaaggaaacttctcatttccccctccccagcccctggcaattccactttctgtctctatgaattggactacttttgacagatacctcctataaatggaatcacacagtatgcatctttctgtgactgatttatttcacttagcataatgtcctcaagcttcatccctgttgtagcatgtatcagaattgccttccttttttaaggctgaaaatcttccattgtgtggatacactatattttgcttatccactaatctatcaatggacacttgagtgcctttcaccttttggctattgtgaataatctgctatgaacatggacacacgaatatcagaggcagccttttcaagcaaagggtttttggggaaaaagccactgtccaggactctaggcttggccactaacttgctgtgtagctgtgggcacattgcttcctgcatcgtgtatggcaattctaactctctccaccttcactgcctactcacagccgtgtgctggggaccagattagaccatggactatgaaactctcagcaaagaaaaagccacgaggggctgttattgttattactcagtggggtcagggcagtggcttcccaaaggcatgagtcactcatggtggaattccagacatcaggagggccgttctgggcagcagagcccagattccagacagagcagtgaccctgacccggagcccctaggggagccacaccctttctctttggccactggctgctgtgaggaaggagtcagtgaatgtcataatcatatgggcacttagggtgagagcctccagtcccactgcctcacgtaactatttaaggaggctcagaaagggtcatgcacttgcccagagtcacacagctagacagtggtggaagctggcctgggtcagatttggacatctacagaagcccttctcctccctgctcgcacccctcttagccccagcatgtgaggaaggcagctgtctccctgagctccgtccttctatgccttgggtttagccatgttgactgctgtaacaaataactccaaaacctcagtggctttgcattataaatgcttggttctttctcacatcaaactgcaataagtcttgacaggagggctctgttttctgcaggtcatatagggattgagacttttcctatttgtggctttcctcattctcagagtcctctccattcagcaggcagatggcagaaagattgtgggtagaagatttttataagccagacctgaaatcagtacaattatttttgcttacatcccattggccagagctcagtcacatgaccacatctaactgcaaagaaggctgggaaatgtatcccacatgtgtgcccaggaagaagaagatggctattggtgagccttggtagtcttccacaagaacatgacccagttctggccaataaaacataaagaaagtatgctgggacaggaggtttgagaagggctggcctcaattattatataaaaaggggtgtggggaaggtcccctattctttccctttaagtggttgcatgaggatgcgatgtctggaactttggcagccatgttgagagcatgacgggccaagcctcagggctacagccaatatactgagggtgctgaagccaaaatgcgggtcctagatgacatcactgaacctctgaatgaaccaaaactggagccacgtaacctccagatttcttgactgcgaaggcacctattattgaattcaggagtaatagggtattctattacttgcagcctaaaacatcctagctgattgacactcaggtgcaaatgctgaaaacagctaagaggacaaggttaagccatgccagctgttacaacgaataactccaaaacctcagtggctttgcactacaaatacttggttcccttgaaacccctcctctgcttgaagttaggtagagccaagtaacatagctttggcctactctggatgttgtgcttttttggggaagttggggacagagcagcagttcaagcacaaaatgacctggctgctttgtgccaggtcctttatacacacagtgtatacacgggagcaaaatgcctggactcaaatcttgagtctgccacctcaccagccatgtgaccttgggcaaagtcaatcaacctcactgagccctagtttccccattgaaaacattggggtgattataaatattctacccacagagtaaaggattaaatgtccaattcagataaagaacttggcacattatctgtaaataaacacttaaaagattctgaccagagcctggtgggatgtgagtaatatcaaccccaccttagagatggggagtctagggttcaaggaaatgaagtccaaggacatataaataataagagacagagcctggattttaatacagacctaattgaacacctgctatgtgccaggcattgtgtgaggtgtttagatatattatcccattgaacatactagcaatcctgcatgggaggtattattattatcattattgttattcctattggacaaatgagaaagccaaaactcagagaagtgaaaagacttgcctacaggccaggtcaagatgcagtacttgaacctaggctgagtccaagcctttattctttccaccatgtataagcctccctaacagaagcccaccagactattatagtggaattgtaggcatcagaggagtaatacatttggctcccatggctattcagggttccctgaagtcatccccaaaagctggctgccagtccagcctgtcaccaaggttgtcctggtgatggctttaccctcactcctccagtagaataactgggccctggagtggatggtcctgagggaggaagtttggctcacttgataaagcagaactttcaaacactttgagctcatccatgatggaataggctgccttgggatgcgatgagttctgtggtcctgggaggatacaagcagagaaagtctggtggccacctgcaaggaagattattaagacagttactgcatagaaagtgaaattagattcaaagacctttcaggtttgaaatctgtggttgcaagattctcaggtcccattttctcagattccagtctaagattacatgatactcaaaatccaggaatctaaggctgcacgagttttctccttggattttttgttccctatttaggcagttagactgcagaacatctactgactcaggaaacagatgtgttagtaaaagcagagaatacatttctgggtttcaaaaacaccccttcctcccaggaaagaacattcctaagagacttgggcatcttgaacacctaatgaatctgaaagaggctctcactttctgtgactgtctttagggactgtccacaaatactctgtttcttttccttttagggtgccttagtctgttcaggctgctacagcaaaacatcttagactgggtaatttataaacaacagaaattcattgctcacagttctggaggttgggaaattcaagatcaaggctccagcagactcagtgtctggtgggagcctgtttcttatagatggtgacttctgtgtgtcctcacatggcagaagggacagatgggctccctcaagcctcttttacaagaacactaatcccattcatgggtggagccctcctgacctaatcaacttccaaaggccccacctcttaaggctatcactgtggggattaggtctcaacatctgaactttggggaacacattcagaccacagcacaggcccatagtaggatttccacttgaactccctcctctgcttgaagttaggtacagccaagtaacaagctttggccaatgaaatgtgtgcagaagtgaagtgtgccacttcctgggggagactttaggagccagtctgtggcttgatgctttctcttgccctctgctgtgcaacagttgaaatggtggttgttctatcagctgggatccaggagcaaggagacacagagcagcgcagcagctgcccagcaggggacgtgcatcaggagccactgagaaacaggacttgagcgttgctgttactgtagcagaactcaccctaccctgactgatgcacagctctcccctcccctccctccttcctcccatctaagaaggctgggaaggaggtcagagaaaaagctatgagtgagcatattttggattttgttggtcagtgggccccagagagctttgaagaattcagaagcagagagcagggaggatctcaagagataaaatggccaagagggccagagacaacctcacgcctagatacaattggggaaaaaaaatgaatggagctgggaaagtgatggggttggggaaaaaaatcccaattgaataagatgaattttctgcccacatatggaatggagcattgaaatgagaatgaatttaaaatagattacatttcca

SEQ ID NO: 2 - DNA, 5748 bp, Homo sapiens
tcaggtcccattttctcagattccagtctaagattacatgatactcaaaatccaggaatctaaggctgcacgagttttctccttggattttttgttccctatttaggcagttagactgcagaacatctactgactcaggaaacagatgtgttagtaaaagcagagaatacatttctgggtttcaaaaacaccccttcctcccaggaaagaacattcctaagagacttgggcatcttgaacacctaatgaatctgaaagaggctctcactttctgtgactgtctttagggactgtccacaaatactctgtttcttttccttttagggtgccttagtctgttcaggctgctacagcaaaacatcttagactgggtaatttataaacaacagaaattcattgctcacagttctggaggttgggaaattcaagatcaaggctccagcagactcagtgtctggtgggagcctgtttcttatagatggtgacttctgtgtgtcctcacatggcagaagggacagatgggctccctcaagcctcttttacaagaacactaatcccattcatgggtggagccctcctgacctaatcaacttccaaaggccccacctcttaaggctatcactgtggggattaggtctcaacatctgaactttggggaacacattcagaccacagcacaggcccatagtaggatttccacttgaactccctcctctgcttgaagttaggtacagccaagtaacaagctttggccaatgaaatgtgtgcagaagtgaagtgtgccacttcctgggggagactttaggagccagtctgtggcttgatgctttctcttgccctctgctgtgcaacagttgaaatggtggttgttctatcagctgggatccaggagcaaggagacacagagcagcgcagcagctgcccagcaggggacgtgcatcaggagccactgagaaacaggacttgagcgttgctgttactgtagcagaactcaccctaccctgactgatgcacagctctcccctcccctccctccttcctcccatctaagaaggctgggaaggaggtcagagaaaaagctatgagtgagcatattttggattttgttggtcagtgggccccagagagctttgaagaattcagaagcagagagcagggaggatctcaagagataaaatggccaagagggccagagacaacctcacgcctagatacaattggggaaaaaaaatgaatggagctgggaaagtgatggggttggggaaaaaaatcccaattgaataagatgaattttctgcccacatatggaatggagcattgaaatgagaatgaatttaaaatagattacatttccagcccatctgaatttcagactgagaatatctgctgcacataattcaagatcccacagtctcaagaggcttgggtcctgggctttgacaatgactcttttcctgggcagaaggttgtacatggacactgggagcacctaggcctggaagctgggagaactaggctctcctgtctgatgtcactttccctgtcactttcccagggaggccttccctgactgcctgacttaaaaggaacttcctctaccaccctggccattctctattcctcttcttaacatcaattgacacaccacaagttttcattttttttttttttttttcttgagatggagtctcactctgtcacccaggctgcacccaggctggagtgcagtggcacgatctcagctcactgcaacctccacctcccaggttaaagcgattctcctgcctcagcctcccgaatagctgggactacaggcacgtgccaccacgtccagctatactgatgtgtttattgtctatttccccacttgactgtaagtttcaaaatggcagatattcctctctctctctctccctcttttttcttttcccttttatttataaaaaacttcaaacatacagaaaacctatcatgaagacccatttaccgcttacccatcatctagatttccaactgttaacattttactgtatttgcatcatgttttttggtgctggcattttctgaagtatataatattcttcactatatttccttttaaaaaattgaagatggccgggcgcggtgtctcacgcctataatcccagcactttgggaggcggaggtgggcggatcacgagatcaggagatcaagaccattctggctaacatggtgaaaccctgtctctactaaaaatacaaaaaattagccgggcgtggtggcgggtgcctgtagtcccagctacttgggaggctgaggcaggagaatggcatgaacccgggaggtagagcctgcggtgagccgagatggtgccactgcattccagcctgggcgacagagcgagactccatctcaaaaaaaaaaaaaaaaaatgaaggtaaggagttttgtctgttgtattcactgccatattactcactgcctggaagttggtaggccttcagcaaatagttgctgagtgagtagaaggcgttaaatcctcatgacaaccctgtgcggtaggtgttattatcccccattttacagaagaggaaactaaggcacagagaggaaaagtaacttccccaaggccacatggttggcaggtgatgaaagggggatttgagctcaggcaggctgagttcagagcccatgcatttagcgcacaattgctctctgcgggcaatggccattcatctccaactgggatgtttattcatcctctttagataccatctacagaggagacccagaggaagaagaggggctcacaggctggccaaaagcaggtgatcttcctctggggacctgatgctctcacaaagcctggggccttctgtcctgccctggggtggagacagaagactccttcccagacgagtgacctttagggtttgttatgaatagagattccttctggggaacgtgatggctgatgctgggaacccgggtccccagatttaacccctaggaatgtggagaggaatctccagacctccacccaggaggccagctctcccagccacccaggccagccagaagagggtggttctaagcagctcttccagttattggaccactgggaggtggactggaaccttccatgtccaggctgggaggcagctcctcagagtaaaaataactctaggcttcaaaatcctggggtctgcctcttcctccccagctatgtgacattcactggacaggtgcctcatgtggggggactttggttttcacatcaatctaatgggactaaatattataccaacctctcagcagggctgggactagggtgaagccagccaggtgctcaaggcataacatttagggaggtgcttgttctgaggcgccaaccctgcacttgctcaggccccggggtgagggcctcggtagatttgcaccctggtcaccttgctgcctcaacctggccccagccctgcctcccagggttgtcgtgggaaggaaatgagatattgtatacaaagcatgttagcacagcatgtagcatgcccttagtgctcacttgtggggaaaattctgttattgttctttttttttttttttttttttttttttttgagagagagtctcgctgtgtcacccaggctggagtgcagtagcacgatcttggctcactgcaacttctgccttccggattcaagtgattcccctgcctcagcctcctgagtagctggattgcaggtgtgcaccatcatgcctggctaattttttttttttttttgagacggagtctcgctctgtcgcccaggctggactgcagtggtgtgatctcggctcactgcaaactccgcctcccgggttcacgccattctcctgcctcagcctcctgagtagctgggactacaggtgcccaccaccacgcctggctaatttttttgtatttttagtagagacagggtttcaccgtgttagccaggatggtctcgatctcctgaccccgtgatccgcccgcctcggcctcctaaagtgctgggattacaggcgtgagccaccgcacctggccaatttttgtatttttagtagagacggggtttcgccatgttggccaggctgatctagaactcctaatttcaagtaatccacctgcctaggcctcccaaagtgctgggctaggattacaggcgtgaaccaccgcacccagcctgttcctattatttttattgactgcctttctgaggttggctgggcctgtttcccagcagtggccctgccttggacctcttgccatggccttcgtctctccctccacttgtacatattataccctttttattatttatccccttgtagcatggtttgattcccattatttactggttccttgtcccatgtctcctcctctgtgtcgacagcctggaaacaatgattgctaatatttaccaagtgctcaccatgtgccaagccctgggctaagcatttacatgctggatttcatctcatctttacaatgatcctatgaggtagggactatgattatacccatttttcaaatgaggaaatggaggcacttaaaaattgagtaacttgcccaaggatgcattgttagaaaaggatggagctgagggtagaatcaagatggcttaatccctaaaacccaagggatggaacccagaacactgcctcttccactcttcaccagcttctgccctgcagggtacacgcagatggctccaagcaggggccccattgctcactgggggaaactggcctccctgagctaagtcaggtcctgggcagagggacagatgctctctgtgcatctctaggccacagcagggcgtttccaagtccttcccagaccagacggcggcttctgctgtaggctatagtaataacaacagcgttgagcactcacactgtaccagagcaggggtggcgccgcgctgcacacctgccgcccagggtctccacagtcctcacgctgcccttgcattgattattgtctttatgtgaccagtgtggtagctcaggtgtcaagacctcaaggcacccagccagggtcgcatctcacgtctatggcagatccaagatctgaacttggacttgtctgaatcctggataagctggggggtgaagctggctgctgaggatcctgtgtgcccctcagccctgttcccaccacctctgtgcctcctccctgctggcagccactgtggccacaatggggttaaccccagaggaaggcattgaaggcgctggggctggggtgggaaggaaggcatatttcggggctccaaggacttgaagcctagctgctccatgcccaggctctgggaccccccaatacatgcacacattgtttaaaatgaagtggaactccaggcaggcaagttttgatttaggggagacagctcctccatggtaatgatactgagccttgttatttgagcaaataggttttctcccagcctctcactcctttctttgtaattcatcttccatcctggccacatgcaggccctgcttggaactctctggggactcctaccccacaggatagtctaaaaccctgccccggtattcaaggctgtttgcagatgttcctcaaccccaccacctgttgctcccaaaattcacacaccccagacctgcacaccacagttgttgctattccacacacaggtcgctgggagcagcgcacggcccagccccgcctttctgcaagtggatccctctgcctggaaagtcctccctcccctcctctggat

SEQ ID NO: 3 - DNA, 24586 bp, Homo sapiens
attacaggcgtgagccactgtgcccttcctaattagctaaattttatgttatgtatattttgctgcaattaaaatttttcaagtgaggtatctataaggaaaggtgagaaaatatgtaagatacaaagataataaaatccagagcaagaacagtatataagtcctgtttccttatgttgaaatatatcaaaatattcaacagaagaccccaggataggaaagatgtgaaattctagactggatcatcaggtccgacggatttacaaagaaggtggccgaggatctctctccccagccttcaccccctcactgactgtgggaaaataaagggcttggggtttggggaggaggtgttgcaggaggagcggcagctccagctatgagacctcacccagagggggccaatactgcccctccagatgccaggcaggggacatggaagggtttggggattcgttgtgggctggggtgggggtagcttgcaggggtctgcttgggtcttgttccctagggcctcctggagggtggagtggtcttagcagcaagaagctggagttggatgttggattcctgagggccgaggaaggacttgcaagggacctccagaaggagaagtgcatcccccccagggtcaagagtgagggagccctgcagcaatggccatctgtgggacatctgtgacactgtcagctggaagccagcaggatggcggcagctcaagtgagacccttcccctccccttactatctccacagcccccacttgtgggggaggggaggaggtccagagaaggagccccccaaactgcctccccaggacaggccccagctgggcaaggggagaaggtttaaacctagatccaattgggagtttggattaatagcttgactggacattttaaatttgagttgagaccatgtttgtgacttaaagtgatggtagaactgtcttatgtaagaattggggccaggcacactttgggagtccgagacaggtggatcacttgaggtcaggagttcgagaccagcctggccaacatggcaaaacctgcctctactaaaaatacaaaaattatccaggcatggtggtgtgtgcctgtagtcccagctacttgggaggctggggcagaagaatcgcttgaacctgggaggcagaggttgcaacgagcagaggttgccccactgtactccagcctggatgacaaagtgagtgagacttcgtctcaaaaaaaagagttggtcccattctccagtgggctagccttggcttgtctcatggtggaggaggctggcgggggtgggtcaggttcaggggggtgggggaaggtggggagcagagggtgggagagagagagagagagagactgcaaggactgcattctttttgaggctcaggctcagaactagcacaaggtcacttccaccacattcaatggaccaaagagagtcccaaagccaacccacattggagagaacgaaggcaaagtcacattgcaaaggggtgtggaaacagatagtggtgcagaatctggcccgctttcataatcagtccactggaagactttgttttcctcgcaaggaaggttggaaatgtagactcactgcttgtccaggcagaagaggaaatgagttcagggaagagcttgccagtccccagcctttgcccagccccctactcatgcacatttaggcacacacctactgtgtgctcagcccagcagggtagattagagagagcgagggcgtcgggatagagggcctgattccccaaccgggtgactatcacttccggtctcatgacctccatgttctcatctgtaaaatggggataaacatcctcatcatctctcctgccattggtatggtggtgacaaaaaacactttatcgattcatgaaagtcatcagacaaagtggatgatgctgtccctgccctcaaaggtgttaaataaagaagatgagaattcaatacatgtccccagctctggtgagactgtaggggttgtgttaacaagggagggagagacatcagagagctgttggcaggggagagccctgtggccaagccttgacagatggtgaacagaatctggaaagacagagggcatggggcatggcagggtgtggaaacagcacacttgcaaaagtgtggaggctggacacatgtgatataaggcagggtcccctaccccatgattcaaagcagaaattcgcaaagactttgatgtaggctgggctgggagttgactacacttgcatgcctgttgcttggcaggatggctttcaaaaaagaaaaaaatataataatgaaagattgaaaacagattattggggagaaaagtatcccaggcgctagacggctgtctctgcagcctctggctcctgtcccacccattccccggccctgacgcaaggctggctggaagaaggtgttctcgagattgttcaggctgagggcctgactggcaggagactgaagcctaccccattcctgcctgggtgccaagctctgcatgaggtttaaatatacccacagcctgacactatgccctagatcatgctaaatgtttccatactccttgaattctcttctcaaggttcatttattgtccccatttttcagatcagtaaactgaggcccagagaggttaactggtttgcccacagtcacacagccagacaagtttgagtatgtctgattctattgccttattccaggtttgggatacaggcagagtagggagaggtttaggatggtaaagaagaatgttccaggaggaacagagttagtgtaagggcagtctaatctagagtcagaatttggagctgtttgttacagcagcatgacctagcctatcctgactgatacaaatcatggtaaactaatttatatgtcctgaaaaatattagaacttagcatctacctcttaggagagcttttttttttttttttaacttttacattttggcaaaacacaccgaacataaaatttaccatctaagcaattttaaatgtacaatgcatggctttaagtacattcacattattgagtttctatcaccatccttccacagaactcgtcatcttgcaaaactgaaattctaaacccattaaggaaacttctcatttccccctccccagcccctggcaattccactttctgtctctatgaattggactacttttgacagatacctcctataaatggaatcacacagtatgcatctttctgtgactgatttatttcacttagcataatgtcctcaagcttcatccctgttgtagcatgtatcagaattgccttccttttttaaggctgaaaatcttccattgtgtggatacactatattttgcttatccactaatctatcaatggacacttgagtgcctttcaccttttggctattgtgaataatctgctatgaacatggacacacgaatatcagaggcagccttttcaagcaaagggtttttggggaaaaagccactgtccaggactctaggcttggccactaacttgctgtgtagctgtgggcacattgcttcctgcatcgtgtatggcaattctaactctctccaccttcactgcctactcacagccgtgtgctggggaccagattagaccatggactatgaaactctcagcaaagaaaaagccacgaggggctgttattgttattactcagtggggtcagggcagtggcttcccaaaggcatgagtcactcatggtggaattccagacatcaggagggccgttctgggcagcagagcccagattccagacagagcagtgaccctgacccggagcccctaggggagccacaccctttctctttggccactggctgctgtgaggaaggagtcagtgaatgtcataatcatatgggcacttagggtgagagcctccagtcccactgcctcacgtaactatttaaggaggctcagaaagggtcatgcacttgcccagagtcacacagctagacagtggtggaagctggcctgggtcagatttggacatctacagaagcccttctcctccctgctcgcacccctcttagccccagcatgtgaggaaggcagctgtctccctgagctccgtccttctatgccttgggtttagccatgttgactgctgtaacaaataactccaaaacctcagtggctttgcattataaatgcttggttctttctcacatcaaactgcaataagtcttgacaggagggctctgttttctgcaggtcatatagggattgagacttttcctatttgtggctttcctcattctcagagtcctctccattcagcaggcagatggcagaaagattgtgggtagaagatttttataagccagacctgaaatcagtacaattatttttgcttacatcccattggccagagctcagtcacatgaccacatctaactgcaaagaaggctgggaaatgtatcccacatgtgtgcccaggaagaagaagatggctattggtgagccttggtagtcttccacaagaacatgacccagttctggccaataaaacataaagaaagtatgctgggacaggaggtttgagaagggctggcctcaattattatataaaaaggggtgtggggaaggtcccctattctttccctttaagtggttgcatgaggatgcgatgtctggaactttggcagccatgttgagagcatgacgggccaagcctcagggctacagccaatatactgagggtgctgaagccaaaatgcgggtcctagatgacatcactgaacctctgaatgaaccaaaactggagccacgtaacctccagatttcttgactgcgaaggcacctattattgaattcaggagtaatagggtattctattacttgcagcctaaaacatcctagctgattgacactcaggtgcaaatgctgaaaacagctaagaggacaaggttaagccatgccagctgttacaacgaataactccaaaacctcagtggctttgcactacaaatacttggttcccttgaaacccctcctctgcttgaagttaggtagagccaagtaacatagctttggcctactctggatgttgtgcttttttggggaagttggggacagagcagcagttcaagcacaaaatgacctggctgctttgtgccaggtcctttatacacacagtgtatacacgggagcaaaatgcctggactcaaatcttgagtctgccacctcaccagccatgtgaccttgggcaaagtcaatcaacctcactgagccctagtttccccattgaaaacattggggtgattataaatattctacccacagagtaaaggattaaatgtccaattcagataaagaacttggcacattatctgtaaataaacacttaaaagattctgaccagagcctggtgggatgtgagtaatatcaaccccaccttagagatggggagtctagggttcaaggaaatgaagtccaaggacatataaataataagagacagagcctggattttaatacagacctaattgaacacctgctatgtgccaggcattgtgtgaggtgtttagatatattatcccattgaacatactagcaatcctgcatgggaggtattattattatcattattgttattcctattggacaaatgagaaagccaaaactcagagaagtgaaaagacttgcctacaggccaggtcaagatgcagtacttgaacctaggctgagtccaagcctttattctttccaccatgtataagcctccctaacagaagcccaccagactattatagtggaattgtaggcatcagaggagtaatacatttggctcccatggctattcagggttccctgaagtcatccccaaaagctggctgccagtccagcctgtcaccaaggttgtcctggtgatggctttaccctcactcctccagtagaataactgggccctggagtggatggtcctgagggaggaagtttggctcacttgataaagcagaactttcaaacactttgagctcatccatgatggaataggctgccttgggatgcgatgagttctgtggtcctgggaggatacaagcagagaaagtctggtggccacctgcaaggaagattattaagacagttactgcatagaaagtgaaattagattcaaagacctttcaggtttgaaatctgtggttgcaagattctcaggtcccattttctcagattccagtctaagattacatgatactcaaaatccaggaatctaaggctgcacgagttttctccttggattttttgttccctatttaggcagttagactgcagaacatctactgactcaggaaacagatgtgttagtaaaagcagagaatacatttctgggtttcaaaaacaccccttcctcccaggaaagaacattcctaagagacttgggcatcttgaacacctaatgaatctgaaagaggctctcactttctgtgactgtctttagggactgtccacaaatactctgtttcttttccttttagggtgccttagtctgttcaggctgctacagcaaaacatcttagactgggtaatttataaacaacagaaattcattgctcacagttctggaggttgggaaattcaagatcaaggctccagcagactcagtgtctggtgggagcctgtttcttatagatggtgacttctgtgtgtcctcacatggcagaagggacagatgggctccctcaagcctcttttacaagaacactaatcccattcatgggtggagccctcctgacctaatcaacttccaaaggccccacctcttaaggctatcactgtggggattaggtctcaacatctgaactttggggaacacattcagaccacagcacaggcccatagtaggatttccacttgaactccctcctctgcttgaagttaggtacagccaagtaacaagctttggccaatgaaatgtgtgcagaagtgaagtgtgccacttcctgggggagactttaggagccagtctgtggcttgatgctttctcttgccctctgctgtgcaacagttgaaatggtggttgttctatcagctgggatccaggagcaaggagacacagagcagcgcagcagctgcccagcaggggacgtgcatcaggagccactgagaaacaggacttgagcgttgctgttactgtagcagaactcaccctaccctgactgatgcacagctctcccctcccctccctccttcctcccatctaagaaggctgggaaggaggtcagagaaaaagctatgagtgagcatattttggattttgttggtcagtgggccccagagagctttgaagaattcagaagcagagagcagggaggatctcaagagataaaatggccaagagggccagagacaacctcacgcctagatacaattggggaaaaaaaatgaatggagctgggaaagtgatggggttggggaaaaaaatcccaattgaataagatgaattttctgcccacatatggaatggagcattgaaatgagaatgaatttaaaatagattacatttccagcccatctgaatttcagactgagaatatctgctgcacataattcaagatcccacagtctcaagaggcttgggtcctgggctttgacaatgactcttttcctgggcagaaggttgtacatggacactgggagcacctaggcctggaagctgggagaactaggctctcctgtctgatgtcactttccctgtcactttcccagggaggccttccctgactgcctgacttaaaaggaacttcctctaccaccctggccattctctattcctcttcttaacatcaattgacacaccacaagttttcattttttttttttttttttcttgagatggagtctcactctgtcacccaggctgcacccaggctggagtgcagtggcacgatctcagctcactgcaacctccacctcccaggttaaagcgattctcctgcctcagcctcccgaatagctgggactacaggcacgtgccaccacgtccagctatactgatgtgtttattgtctatttccccacttgactgtaagtttcaaaatggcagatattcctctctctctctctccctcttttttcttttcccttttatttataaaaaacttcaaacatacagaaaacctatcatgaagacccatttaccgcttacccatcatctagatttccaactgttaacattttactgtatttgcatcatgttttttggtgctggcattttctgaagtatataatattcttcactatatttccttttaaaaaattgaagatggccgggcgcggtgtctcacgcctataatcccagcactttgggaggcggaggtgggcggatcacgagatcaggagatcaagaccattctggctaacatggtgaaaccctgtctctactaaaaatacaaaaaattagccgggcgtggtggcgggtgcctgtagtcccagctacttgggaggctgaggcaggagaatggcatgaacccgggaggtagagcctgcggtgagccgagatggtgccactgcattccagcctgggcgacagagcgagactccatctcaaaaaaaaaaaaaaaaaatgaaggtaaggagttttgtctgttgtattcactgccatattactcactgcctggaagttggtaggccttcagcaaatagttgctgagtgagtagaaggcgttaaatcctcatgacaaccctgtgcggtaggtgttattatcccccattttacagaagaggaaactaaggcacagagaggaaaagtaacttccccaaggccacatggttggcaggtgatgaaagggggatttgagctcaggcaggctgagttcagagcccatgcatttagcgcacaattgctctctgcgggcaatggccattcatctccaactgggatgtttattcatcctctttagataccatctacagaggagacccagaggaagaagaggggctcacaggctggccaaaagcaggtgatcttcctctggggacctgatgctctcacaaagcctggggccttctgtcctgccctggggtggagacagaagactccttcccagacgagtgacctttagggtttgttatgaatagagattccttctggggaacgtgatggctgatgctgggaacccgggtccccagatttaacccctaggaatgtggagaggaatctccagacctccacccaggaggccagctctcccagccacccaggccagccagaagagggtggttctaagcagctcttccagttattggaccactgggaggtggactggaaccttccatgtccaggctgggaggcagctcctcagagtaaaaataactctaggcttcaaaatcctggggtctgcctcttcctccccagctatgtgacattcactggacaggtgcctcatgtggggggactttggttttcacatcaatctaatgggactaaatattataccaacctctcagcagggctgggactagggtgaagccagccaggtgctcaaggcataacatttagggaggtgcttgttctgaggcgccaaccctgcacttgctcaggccccggggtgagggcctcggtagatttgcaccctggtcaccttgctgcctcaacctggccccagccctgcctcccagggttgtcgtgggaaggaaatgagatattgtatacaaagcatgttagcacagcatgtagcatgcccttagtgctcacttgtggggaaaattctgttattgttctttttttttttttttttttttttttttttgagagagagtctcgctgtgtcacccaggctggagtgcagtagcacgatcttggctcactgcaacttctgccttccggattcaagtgattcccctgcctcagcctcctgagtagctggattgcaggtgtgcaccatcatgcctggctaattttttttttttttttgagacggagtctcgctctgtcgcccaggctggactgcagtggtgtgatctcggctcactgcaaactccgcctcccgggttcacgccattctcctgcctcagcctcctgagtagctgggactacaggtgcccaccaccacgcctggctaatttttttgtatttttagtagagacagggtttcaccgtgttagccaggatggtctcgatctcctgaccccgtgatccgcccgcctcggcctcctaaagtgctgggattacaggcgtgagccaccgcacctggccaatttttgtatttttagtagagacggggtttcgccatgttggccaggctgatctagaactcctaatttcaagtaatccacctgcctaggcctcccaaagtgctgggctaggattacaggcgtgaaccaccgcacccagcctgttcctattatttttattgactgcctttctgaggttggctgggcctgtttcccagcagtggccctgccttggacctcttgccatggccttcgtctctccctccacttgtacatattataccctttttattatttatccccttgtagcatggtttgattcccattatttactggttccttgtcccatgtctcctcctctgtgtcgacagcctggaaacaatgattgctaatatttaccaagtgctcaccatgtgccaagccctgggctaagcatttacatgctggatttcatctcatctttacaatgatcctatgaggtagggactatgattatacccatttttcaaatgaggaaatggaggcacttaaaaattgagtaacttgcccaaggatgcattgttagaaaaggatggagctgagggtagaatcaagatggcttaatccctaaaacccaagggatggaacccagaacactgcctcttccactcttcaccagcttctgccctgcagggtacacgcagatggctccaagcaggggccccattgctcactgggggaaactggcctccctgagctaagtcaggtcctgggcagagggacagatgctctctgtgcatctctaggccacagcagggcgtttccaagtccttcccagaccagacggcggcttctgctgtaggctatagtaataacaacagcgttgagcactcacactgtaccagagcaggggtggcgccgcgctgcacacctgccgcccagggtctccacagtcctcacgctgcccttgcattgattattgtctttatgtgaccagtgtggtagctcaggtgtcaagacctcaaggcacccagccagggtcgcatctcacgtctatggcagatccaagatctgaacttggacttgtctgaatcctggataagctggggggtgaagctggctgctgaggatcctgtgtgcccctcagccctgttcccaccacctctgtgcctcctccctgctggcagccactgtggccacaatggggttaaccccagaggaaggcattgaaggcgctggggctggggtgggaaggaaggcatatttcggggctccaaggacttgaagcctagctgctccatgcccaggctctgggaccccccaatacatgcacacattgtttaaaatgaagtggaactccaggcaggcaagttttgatttaggggagacagctcctccatggtaatgatactgagccttgttatttgagcaaataggttttctcccagcctctcactcctttctttgtaattcatcttccatcctggccacatgcaggccctgcttggaactctctggggactcctaccccacaggatagtctaaaaccctgccccggtattcaaggctgtttgcagatgttcctcaaccccaccacctgttgctcccaaaattcacacaccccagacctgcacaccacagttgttgctattccacacacaggtcgctgggagcagcgcacggcccagccccgcctttctgcaagtggatccctctgcctggaaagtcctccctcccctcctctggatcctcctgggtcaggctgggtgctcctctgaactcccaggctgagggttgctgtgtaatttgatactacattgacattgcaggaagatcatgtatggctgagtagctaaaaatgcaggctttgaacttggatgtgggttcagcctcagctgtatctcccgccagctgtgggacattgggctggcgtctctgagcctcagtttgcttctctgaacatagaatgatacgccctactccattaaggtgctgagggtgaaggaaaccacgggctcagtgtgggcagcttggccagggctccaagcgcatcgggtgttcatgtagtccttctagtgccaggcggtcattagcaacttggtgccagtctctgagctggtctccaggacggagcagtggagggaccatgtagcccctgctcccacaaacacagacattggacagccaattagttaccccagttcgttaccatggagactataattagggattatagtcaccctgcccaagcgcacaggcctcacctcccatccttgccttagctttgaagctccctggagcaggatctaaactggatttgtctctgtaacctcagttcctcattattcatggtcggaatgctcagcaaacgtttaagtggaagagatttccataacaaacacttgggagttcagaggagcacgcggtccaacctgaacagagcaggaggatctcagaggagggaggccactaggtaggatgcggcggcactaagggtagcacttagtttgtgacaaggactgttccaagcacaccacttggatcatctattaaattctcacttatttatttatttattttaaaattgtgtttatttatttatttatttatttatttatttgtttgttttgagatggagtctcgctttccaggctggagtacagtggcacaatcttggttcactgcagcctcttcctcccaggttcaagcgattttcctgcctcagcctcccaagtagctgggattacaggcatgtgccaccacgcccggctaatttttgtattaagagatgaggtttcgccatgttcaccaggctgatctcgaactcctgacctcaagtgatctgcccgccttggcctcccaaagtgctaggattacaggcttgagccactgcgcccagccagtgatcacttatttagatcacttactaaaatcatttaattatgtcaacacctctgtgaagtatgtactgttatcaccattcccatttcatagatggggaaactgaggcacagaaaagctaagtaaactgctcagagttacagagcctgcgagggccacagccagaattcaaacccaggccatctgcctccacagtccactttctatgtccctctcccgagatgatgtccctttcccaggggtgtctggaaagggtctggcccctggtcccagctcaagcagctgtccagggaagcctgaagacctggcccatctccactgcccaccgggcttctctgcgctccacttcccaggtggactgtggaggcaaataaggccccagctgcagcctctgaagactcctgccaagctggcactttgaggcctgggggtgtcccaggggatcccagcccagcagctgggctgacctcagggccagtgtttccgtaaacacccggagagccagccccacgtggttgatctgtgggttgctggccaagaggggctgaggtttggctgacctcgtgcggtttctttcaacaaggctacttccaccccctccgcctggctgggcttccagtaatgaagtgttttctctggggctaggggagctgatggggctggtggcgtggggcactggggtcttcctgtcccacgtgccctccaccctgggcttctggaagctggtctagatgcccctagctgccgcctgggcagcccatatgcccacgccggtccctgatagtgaactggcccgtaaggggaccaggtctcgggatctgagcatggagcaggggctgcgcccaggagatagggtgtggctagactttcccctgctggtcctttccggggatctgaggggaaacttctcctggggacacacccgggtagctcagagatggaagaaaaggtctccattacagctgccacctcttccccacccaaagagagtgtccgcagggggccgtggggcaggagtgagtactgaaggaatactaaccacgatcactgctaccatctcctgaatgtcactgccccagccctttaattctcacaacaaaccttggaaactgaggcttagagagaggaagtggctggcccaaggtcacatagtgagtaaatgagcagagcttctccccctttcccttgaatcacctctatcttcctgtccagatgccaggcagcaggaactagcaggtgcttttgggtcatcttttaagaggcaatatagcacaatgagtgagagcagggactcaagggccagccacctgggttcaaatcccagctctgcttcctactggctatgtgaccttgggcaagtcactcaacttcttggttcctcagtctccccacctgtataatgaggataataatgatgcctcctttagggggtttctgtgaggattgcatatacacgtgacacataataagccctgtgccatgctagttatcccagcctctcactcttcccattgaaaaggtgaagacacagacccagagatggaggcaaattctgcaggggtcatgcccggggcagagcatggttcagctatgtctcctatggtgctgccaaggagccaccatgggcttgagctgagaggagccacctggcaccggacacgtgacctcctcgagggaagggaggctctgcagagagcaggggatggtggaggagcctggctttatcttccatccttcaggagcggggaagggcagtgtcagagccaggagaggagagaagcgaatgaacgtgctgtgtgagctccagtcagtccctactgactctgggcctgtcactcctgctgagggactcgggtgtttggacttttagacttggaggggctcctcggtggggccttgggggctgctctgggtgagggctctcaccatttgcttcatcccaaaccactgtccttgggcctgttttaaatattagagtgtagcatggggttttgctgctctaacaaagggtcagccatcttgagaaggaggctctgtgatgagcagggaatggggctcccctgcccccccgagaccctggggcccaagctgatgactggccagtgactcactcccttctcagcatgtcctgtcatcccatgactgggagcccctcgggggtggctcctaaccaaggtccccctgaccaaggcctccccccaccctccccctaacacacatagagactgggaacaattaactccctcctaaggccagaccagatgttcacgtgggcattggttttgttgaccacatgtgactcaggagctccctcagagctggaagagtcccaagaggctaaaagggcaacctgtcacgtcacagctgggaaactgagtcccagagaagccaggtgagttgcctaacatccctcaggggtagaagggaggaaggaacctggagttcccatgcctgacccagaggctttctacctctccaaatagttctcggatgtgcccaaggcctcagtccccattcctacctccagttgcaaatgtcctccccaactacacagagcctctcagcttcatcccaccccacctccaactggctctcatggtttcatccaggctcagctacttgcagctccccaaatagctcctgctgtcaggccacctccaggcctttgtactctcctgctgctctgttttattttcctcttcacctggacaactcctaatcttgctccaagactcatctcaggtgtcaccttctccaggaagcctttcaaaaccacctcctccacctcccaggctgggttaggtcctccatctcttcaccctcagtacctagtatctcccacttactgtgctggaatcatctctttgcttgtctctatattgccctctagtctgtgagctcattgtggacagagaccttagtttttattcttaatagtagggaatgacctattacattcggtgtttgctgaatgaatgcataagtggatggatggatgaatgaatgaatggttggatggaagaatagatacatggatggatggattgatggatggatggaatgagtgaccaaatggtagatgaatggacaaatggaccgacaaacatggaaggatggatggatggacagatggattgatggacaggtggattgatggacaggtgggtcgatgggcaggtggatgaataaatcaggcagataatggcatctgtagggactcagacagtgagggctaagtccctggagcctggatatcctgactgatgaaggtgctcttggatgggaagggaataacctaacctgttgtcttcctactccaagagatatttggtccagaacaaagccacccctgccctggtgcctgctcccttctgaccaacaggttccaactcagtggggtctcctgaactctggtaactcatctgacaccagagcctataggaatcaccctgtctctgacattcagggattctgcattcctgaggccctccctccctgcctctcttcaggtcagagctgccgccccataaatgctttcaagcatagaaacatacacccctagagccaggaagttgtaaaaatgatgggattcacccctctaccatttttgcagatgaagaaactgaggctgagcaaggccaagaaacttgcttaaggacacacagcaatagagctgggataagagcttgggtctttcaattcgtttattcgttcatacagcaagtatgtatctagcgcctaaagtgccaggctcagtgcctattcccgggcatgctaggcctgtgcataagctttcatgttaatttaaaagctatttccatcctccatatgacctcctccagctccccagcaggctggtctatgcctcactagctgcatgcctggcatgatccctatgacaacaccctctcccagcaaatgaggaccacttcattgtcaggaagcctggctgggactggtgtgtgctgccgtgtgcagaggaggcagtcacatgtgtgtgctgtgagctgcacattccatcctagccttagtgaggaccgtattagtccctgcacgctcatccttgccagctcagactggagccaagcattaaactgttcaagccccacagctgccccaggcgagccattgcatggcacctgggagctcagggccaggagcagacctctgaattcctgcccaaaccagggaatatgtggtgagaggaggtcatagggaggtgcctgggggctggacatttgcaagccagctgagcaggcagtactcagcactttcctcttcacccctcccaccatggcaaaggcaggggcagcgtgggctagccagccttggagagatggagcctcaagtctaggggcagcagcccagcctcgggcgagccagggctatttgctgggccttctatgaggcttccatgaagtatgtaacctcgccgaagacatggaactactcagagtcattaagagccaaagaaaggctcagctgcgtttaacagaaaagcttctgggaacaaatcaatgaattggagaacaaaggaagactgcagaagacgaacagaaccagaagccatgtctaggatgaaatcaacatgaggtagagaatcctgatgacattgatcaggatgaaagaagtatgaggcaagggagtaaaatcaaatgccgagtaaaaagggggaacaacgttgaccaaggaatttgaagttaatttaagagctgttatgaacaatacaaaaaagaaaattataggcccatttcacttatgaatatatagatagaaaaacactaaacaaaatatttgctgactgaattcagcagagttaaaataatgacaccacatcaccatcaggaagcgtttatcccggaaaaacattccagaaaatccaccagtgtaattcactacatcattagatccaaaggaaaatctatgatgtcaattgatgtggaaaaattttttgataagttccttttgtatttatgatgcttacaaatttgaaaattctgggaaaatggagaaattaatagaaaggtataaaatgtcaaaagatgggcccaagaagaaatagagaatttcagtaggtcaatcagtattacagaaactgtaatggtgtcaaagccctcccactcccctaaaaatcagcctagatgttctcatgggtaagtactgctgaacctttttttttttttttttttttttgagacaaggtctcattctgtcgcccaggctagggtgtagtggcccaatcctggctcactgcaacctctgcttcccaaggctcaggtatcctcctgcctcagcccctcacgtagctggaactacaggcatgcaccaccacacccagctaatttttgtatttttagtagagatggggttttgctatgttgcccaggctggtcttaaactcctggactcaaacgatccacctatctaggcctcccaaagtgctgggattacaggtgtgagccaccgcgcccagcctgcagaaactttttagaaacaattaattcgtatcatatgcaagttgcttaaaaagaaaacaaaagaaaaaaaaaccaacctatcttattttaaaagtgttgtcttgattataaaagccagataagacaataccacaaaggaaagtataggtccatttcacttatgaatatggataggaaaacactaaacaaaatctttcctgactgagtctagcagagttaaaataatgatactacatcaccatcaggaagggtttatcccagaaaagtatccacatctgaaaatccaccagtgtaactcactacatcattcaatcaaaaggaaaaatccaacgatgtcagctgatgcagaaaaaggttttgataaggtctttatgtatttatgatttttaaaaattcttagcaaactaggagcatgagagaagttccttaatttagtagggatttttaataccaaaaacctacagaaaatattgctagtggagaaaagttttatataatacatgccttttaaggtgaggaacaaggcaagaatgctagttattactgctactgtttaatacatagagctggagagctgggctgagctacaaggaaagaaaataagaggtgtaattattggaagggaagagataaaactgtcattgtttgtagatggtgtgatcatctaccttgaaaaaccaaccaaataaactgacaaaatattagaacaaataagagagttcagcaaggttgccagatacacagtcagcaacaaaaatcaatgacgcttttacatcagcaataactaaccagaaaaacacaacataattttgacttaaatagaaaggttttaaaataatatatacatataaatatattatatataaaatgcatatacatatatatatacacacatgcacacattttaaaagcacagctggctatggtggctcacgcctgtaatcccagcactttgggaggccgaggtgggaggactgcttaagctcaggagttcaagaccagcctgggcaacatattgccaaaattttttaaaaaaacatttagccgggcatggtggcacacacctgtagtcccagctactaagggggctaaggtgggagaactgcttgattccaggaggtggaggctgcagtgagccgtaattgcgccactgcactcgagcctaggcaacagagcgagattctgtctcaaaataaataaataaataaaggtatatatatacataagtataaaaatagcgtatatatataaaacattatatctctctctacacaccacacacacacacacacacacacacacacacacattattatgtttctaatcacatgaatgaaatctacatgtagggtgcatttggcagctctgggtgtcatcagggatctgagttcctttatttctccttcgccctcttctgcacacgaagtccatcctcagggtaccctcatggtccaagatggctgcagaactccaccatcacgtccgtattactgactggaagcaggaggcagcaatcagtggtggtggagtcaccaaagggaagcccttccttttaaggagcctttccagaatcggcacacaacactcctgcttgtatctccgtgctggaacctatcccgtggccccgcctcctgcaaagctgagtgcgtcgccaccccaaacaaaaaaatcagtgtttggtgactgagggaggagggaagaaggatattggaatgggcattgatcaggctctgtcacagatctcagtctccaaaacacgaaactggggcactgaggtccagagaagtgagggaatttacacacagccacaaagcaaattagcagcggagttgggattttcacctgactgttgaccttcccatggtacaggtgtcccctcacaccctggtacatccagccactacagcactgcccctcctcacttccagccctgctggggtcaggatctgttttgtatttctctgtccccactacctaatgtcacacctgtgagctccacctccccagcgtcggcttgggacttggcatggggtagaggccgtaagcgggaaagcgggcacacacctcgggagctgacaaactgcaaagggctttcaaccgcagatatttacttgtggcttccatatgctgtaccttgatggtgatgtttcgtaagtttcacttttcagatgcattttttttttttttttttttttgagatggagtctcactctgtggcccaggctggagtacagtggcgcgatctgggctcaccgcatcctccgcctcccggtttcaagcaattctcctgcctcagcctcctgagtagctgagattacagatacgggccaccacgcccagctaatttttgtatttttagtagagacaaggttttgccatgttgtccaggctggtcacgaactcctgacctcaagtgatctgcctgcctcggcctcccaaagtgctgggatgacaggcgtgagccaccgcgcacggccagatgcatttcttagacgctaaaaatgttcagcctggcccaggcctggaagaacatgcaggccgcttttatttttatttttttttaacagatggagaaactgagacccagagaagcaaaagtgtgtgtcccagatgccaaggtacctgcggcaaagaatattacctagatgtccctcactctggttctccttcattgatacacatggaatgatggtatttccccgccttccttgcagttaagttggggccatgtggctagctctgactaataagatgtgagtagaagtgatgatgtggcttctccatccctcttttttcctgccaaggtgaccttggaggccaccggtctagaacagggattcacaaactgtaatgtgcatgcaaatcacctgggggtcttactaaaatgcagatcctgatagtggggtctgggagtctgcatttccaacatgcaaccagctgatgctgatgccatcggtccttggaccacacacttgagtagggaggagctacaggatgtgcctggcccactttggaccattcacgagcaagaaattagcttcactgggttaagccactgagatgtgggcattagtttgtgatctcagcacagtcttacggaaattgtcatttagccatcaaccaacattgactgagttcctaccatgaactcctgtgtgacctgggtgcctcattctgaatgaggtgctcactcttggggttgtgcaagtgcaaggtcagcagctgagaatgagagcctccctaaatgttatacccgacatgcctctgtcacctcaccctggtcccagccctgtaagtcggtagcgggagccgggatttgaagctcggacctgttgacttctgagcttgtgcttcctcctgggaaagcaaaggacagccacactcaccctgggcccttgtgtgggggctgcggctgcagccaaaagactcatgggttccctggatgcttatatccctctggtgccaaaattggacagtttgaagggagggctgaaccgcagcaaaccaatcagcaaagtggcagctcccaccgctcctgccacacccactcatgctgaactgtgtgtgcaagctccatccctcacacttcatcaccaaacacccttgatgatgacgcctgcttcctgatctggccaggccccagggcccctactgcccacactttcccatcctcagttatcagacagaaaaagttccaagaaaaatccatgctctgactcagagggccctaggtgggcatagcactctgcctcgttcttgccacctccctgccccgtatggccctgtcttcttcaccatacgtggcacccatggcccacctcacctcctcattgtcaaggtctccttgctctgctatggacatggctgggaccagcgtgtctccctccaactctcttcctcacacctcctcatttctcccgtcttccttcttgcctcagagatagaagtggcttaaaactgttcctttcaggaacaactaatcagtggccacagaggtcagaatagcgggtacctggaggacagagggtagagtcttggaaggggcataaggaaacttctggaagtgtagcttgacctgggtgattatcacatgggtatatacagtcatgtatatacatatgtcaagagtcaaaattagccaaacatgctgcctcatgccaccagctactcagaaggttgaagagggaggatcccttgaacccaggaggctgaggctgcagtgagccatgttcatgccattgcactctagcctgggagacagagtgagactctgtctcaaaaaaaagaaagaaagaaaggaaagaaagaaagaaagaaagaaagaaagaaagaaagaaagaaagaaagaaagaaagaaagaaagaaagagttgtcaagctctacacttcatattagtgcactttaagcacttttctgtatatacattacctctcaacttaaaaaacattatcacagagagctctatggacagtagcagaaataaacagcatcaaaaactgaaacttgggtgttggagtcatatgaacccgcactgaaaacctggctctgttttctagctgtgtagctttaggcaagttacttaacctttctgaacctcacttttttcaattgagatgtggatcatgaggattagaaatgctgctttttataaacagtgcttagcacaagggctggatcttgctgggtgctatacacaattgcttttatttttattaatatcagtggcctagggaggacaggaaagtcggagtgacctttcctggatgcaggcaataacgggtggggggcctacagaatttaaagataaaataaaactgatgagaagtcagtctgcttttatgatcactgtgcaatggcagatctaaataatttcagtggtaaaatactttgtcctgaaaataccctttattgatctaagttctaacaattggtgcagtaactgttggggtttaataatgtatatgtaaagcttcaaatcagcacatttttattcttatcctttaataaacatattctacatggaagtcaacttgacttggagaactttaagaatcctatagttgcccccagagcatgtggtctcaggaacacacatcagttgagagtaagctcctcacaactctggaatcttccaagcttgctttgaatgcattcctgtctccaccgtccagcattcatatttctgcatttatttttattattattttgtgtgtgtgacagagtctctctctgtcgcccaggctggagtgcagcggcaagatgtcggttcactgccacctccacctcccgggttcaagcaattctcctgcctcagcctcctgagtacttgggactataggtgtgcacccaccacgtccggctaatttttgtatttttttttttagtagggacgggtttcaccatgttggccaggctggccttgaactcctgatctcaggtggttctcccactttggcctcccaaattacagacgtgagccaccggcccagctgtatttctgtgtttaaacagtagagtgaaatcaactatgaacgcagaatgatgggaaagatgacgataagggtatttcaattttgtcattttacgaaactacttggagttttgatttgtatttacagtttttaaaagagtaaaacagtgtgaactgtgaatggtaatgattttgtttggtaagtgcaaattttaattcatacatgaaaaatatttgttttgtttcatgattattactgaaaataattttgtactatgaaggaagaggggtgttaaaaatgatccactgtggatgtaaattattctaggcatgcttctgactaaaacattagcatttccacaagaatcccaaaaaataaaacaaaatttaaaagatcccttctgtttcttttcctccaagtttccagacccccatctccaccctggccacctcttcctgccataaataatcaaatcccacactttcatcttcaccttccgtttccattgcctcttccgatgggacagcacccgtggggaatctcctccatgctcaca

SEQ ID NO: 4 - DNA, 34429 bp, Homo sapiens
gtgatgggagcaagcttcctggatttccgagccttggtcataaagaagctttgtggtgtcctttggggcctcttgaacattctctctgggaacccaagcttctagaagagaccatcatgctaagagagtccacatatggccattccagttgacagtcccactgagcccaggcttccaccatccctacgaagacagcaatcatgttagcgaagctgtgttgggccatccagcccagctgcccactgaaaaccaggctttggtcaatgccatgtgggacagaagaattacccaagtaagcccagcccaaattcctgacctatagtattgagatatgtaatgaaatggatgttattttaagccattgtgttttagggggagattgtcacacagcagtaggtaacaggaatgcttgcttctacctgccccagccctccagcctctgcaccttagtcacttccatcctgacacctggaaaaccctttacccagatcctagactatcaaaattctgcattccaaatgggtcagatccaaagggccaggctgcgtgatgcagttcttctgtttgcccctgcaggtgcactctccacccttctgcacgctgctctgctcctctgtgtccggcagccatgctgctgtgggtgagaccaatgggctctcctgccctctggctctggttgggttttgtcaacagggagcaccagcaggagaacagcagatgagaggagagaggtcaggatattcattccccctttccctcggtgcacagtcactgggctgactgtgtctctctaccaaggccacatctcctgtcagtcctcctggcccacctctccataccctccccattccagattccctcttgcctattgattgattgattgattttgagacagagtctcactctgtcgcccagggtggagtgcagtggtgcaatcccagctcactgcaacctccacctcctgggctcaagcaattctcatgcctcagcctctggagtagctggaattacaggcacccaccactatgcccggctaatttttgtatttttagtagaaacttggttttaccatgttggccaggctggtcttgaactcctgacctcaaataatccacccaccttggcctcccaaagtgttggcgttacaggcatgagctaccgtgcctggcctcctgccgttttcttgaaaggcagtggttccctttgttaccagagtcccacgccacccgttgttgctttccttaaactctcctcgctaggttcaggtttccccagaagcagagcctgagacaaagatttcaatgcaagtagtttatttgggaagaggaaacatgggaaggatgtgggtgcgaaacaagacaggaaaggggaagaagctgacatgagcaggtcaccacactgagcacctggagctctatccctgggcagcactctgggagatgatgaatatgttgcaggcttaacccagcagaggagcgaggaagctggggaatctaactgccccctcccctctggcaatgcttccaggacattaacttcctggcactcttagtttgttcaacatgaccggctgagtttcttgcatggctagaaaatatttgcagcaatgagagagagactctgttagcagtaagtagctattgccatgtagaggtgattttgagggcatatgggcagctacaccagcccacacctatgtaaataactcccatattaaaccctcttcaattactcagtttgagtgtggcacctggttcctgccaggaccccgagtgatacaggctggtcttgagcttcttcatagcaatacagagtggaccagtgactacagaaagcttgagaggggctggagagagatgccttccccaatattcattatccacacagcacgccactcctgtgagaagacaacagagattgtgtatgtttgagaatgtctctctacctccaatgtagccctcctgaaaaatctagttcaagatctattccaggccaggcgcagtggctcacacctgtcatcccaggactttgggaggccgaggcgggcggatcacctgaggtcaggagtttgagaccagcctggccaacatggtgaaaccccatctctactaaaaatacaaaaattagccgggcatggtggcatgcacccgtaatcccagctactcgggaggctgaggcatgagaatccctctgggccacagagggagactctgtctcaaataaataaataaaaatcaagatcaaaatgtatatgatcaggagcctcagctccaccacttacagctctgtggctttgggaaagttgttttgagccttgattttctcatctgtgtagtggggataacatatacatactaattaataggataaaccatagacacgcctcgctcataggaggagaagaacatcctcacacaatgggagaggtggggattgtggaaaggagagagcaaatgcctcgtcaagatgctgctgtgctgaaacataaatccagtgttgccagatcctccaatcatccaaaaaagccggagacccatcttttaatgtttaaactgtattcaaatgtgtcctaatgtttaaaactttgtataagccaaagaaaacatctgtgggccagattttgccccacacagccaaggtccctgctgattctgatcttctaagatctctgaataagaaagaggacaagggacaggttgccctttcactcacatttatcagacaggattaggatcagttgcacacaacagaaaacacccaaataatagtggctgaaaaaagacagaagtttatttctctgttgtgtaaaaaggccagaggcaggcaatgccactgatgtgacaactctgtgaagatgcctccttctatctctctgctctgccatccctagcatccagcccctatcctcattgtgcagtatggctgctggggcaccagccttcacatctgcagtccagagagcagggctgaggaaaggatgcagcagctagtgcttgtctctctttttttttttcttgagacagagtctcactcttttgcccaggctggactgcagtggcactatcttggctcactgcaagctctgcctccggggctcacgccattctcctgcctcagcctcccaagtagctgggactacaggcgcctgccaccacgcctggccacttctgtcttttaaagatctagatacctggttttcctcacaacaaattctgcttatatagtcacatggccacatctaatcgcaaaggaaactaggaaatgtcttatacctgtaaggcaaggtacccagctaaaaaaaaggagattgtgttactaaagaagaggatagtaggcccactgcagtggctcatgcctgtaatcccaacactttaggaggtcgaggtgttcgatcacaaggtcaggagttcgagaccagcctcacgaacatggtgaaaccccgtttctactaaaaatacaaaaattagctgggcacggtggtgcacacctgtaatcccagctaattgggaggctgaggcaggagaattgcttgtacctgggaggcagaggttgcagtgagccatgattgtgccactgcattccagcctgggtggacagagcaagactccgtattgggggaaaaaaaaaattagaggatagtagatctagaaggctgctcatttctgccacatcaaatagcctggtaggtgaggagggtatatggataggtggaaagagtgttaccaggaagccagattctgctgtccatatcatatgtctttaagcctctttctgaccaggagaagaaaataagagagcaagatagaaagaggcctgagtataatcatagagacaacttaccaaggacctgttgcatgccaggcccagcactgagtcttgtgccaacattgttttagtccattttgtgctgctatagcagaatacctggaactgggtaatttttatggaacagaaatgtattggctcatggttctggaggctggaaagtccaatatcaaggtgctggcatcattcaagggccttcttgctgcatcattccatggtagaagatgagagagtccgagagggtaagagagggagcaagagattgatctcacggcctcaagcctttttatactcagcattaatccacccatgagtgtggagcccccatgacctaaacacctcccatgaggccccacctgccaacactgttgcattggggattaagtttctaacacatgcttgttggggaaccacattcaaaccatagcaaacatcatctcagattattcttttcatccagcctatccggtgggtgggcctcgtgttattgtggggtggggtcacatcttgcctgtgccagctggggtaggaggcctggacatccaattgtctcccagattgataaccaacccacccttctgtcttctgccctacctgacaccacttggtcttcagagatttctggtccctccaatccctgagcctgagattctgcaatttgctttgtcctaaaggctccccgtgagcagccaggtttcaacttcctgggtttcttgtcagtccccactcaccatctgccttccagcttccggaatttggttgattcttctcatctgctattttcttcctcatacgttttctttgtcccagtagatagatgtgcatttaaaaaaaaaatccctgtgtcattttcttggaatttcagagaacaatggagagaaataagtgtgttcaacctgccatgtttaaacagcagtctccagcctcagttcttgactgggggaatcctcagccctcaggaggattgtatggtatccccatccttcccccattccttccttatcctgctccaggagtccatgggagccctcggcacacaggactctcttccccactctctgaacctggggcatagttctgtcctgcctccatagcccatacctgcttctcaagagcaggggccttgtcttcttctctctacttcgacaggtctgggcaggcctcaggaagatagatatgagctcatggtgtgggtcattcctaagaagtcactttggactttgaggagttaaaattcaaagctggggatgagagtcaggcatttctaaattagaatatcaagtgtattcccactgtatttacaatggaggccagcatcaacactcaaggtgaaagcctgatagagtcacattggtccttgaaaacctcttaggaagatgccaggtggagacagaggcatcgtccctcactgaatctgatacagccagcattttctccggggcttcttccccatgtcttgagtaagtgcctgctggagatcctggtttgggttgagaagctgtgttatgtagacaaagtgcatcttcagatcctagaatcttcctcagtgggtcatgagcctcatgttgctcataggaaaagaggccaagaactagggtgaccaaccatcctggtttaccaggtctgagtagtttattgaaatacagagttttcagtgctaaaaccaaaacagtcccagggaaattcccaattgtggtcaccctacagaacaaccgtaacaacaggattacctctcacacaccctcctggacatgtgcatgttacacaatttgtccactttctgttgctgtcatagaacccatgggactgggtaattgacaaagaaaaggggtttgttttttacagttctggaggctgggaagtccaagacagggtggctggatctggtcagcttctggtgagggcctcgtgctgtgttgtaacacagcagaatgcatcgtagggtgagaggaagcaagagaaagccgaggaagcaagagaaagccgaggaagccaaactcacttttgtaatgaactgctctcaataactcacccacttctgtgagaattaacccactcctgtgagaaaggcattaatccctcctaatgacctaatcccctcttaaaggccccacctcccaataccattacattggggaccaagtttctacatgcattttggaggagacaaaccacatccaaaccatagcacacacacaacataaaatcgttatctcctacagtttaccacacccctcaacctccacgcccctctcaccagccttttttttaatacgaattcttgctgttgttggcctgggctggagtgcaatgacacggattcggctcactgcaacctctgcctcctgggttccagcagttctcctgcctcagcctcccgagtagctgagattacaggtgcccgccaccacgcccacctaatttttgtatttttaatagagatggggtttcaccatgttggcagggtggtctcaaacttctgacctcaggtgatccacccacctcagcctcccaaagtgctgggattacaggtgtgagccactgcgcccggcctcaccagcccttttaagggaaatagatggtagacttgttcggagagtgggctctggaactaggctctggaagcttcagttgcagcattcattagctgtatgtgtttgggcaagtcactttacctctctctgcctcagtttccttatctataaaattggaagaataatagtaagttctactctgtcaggtcattgtaaggattgaatgaattaatattatggagagcagttagaacagtgcctgtcatggaggaagctacacaggtcacaactccttaactgaaactccagtgtctcaggatcctgatgcattttggaatttagggagttttgggattttggaaagcacatgacttatataacacactagtgggtagtgggatctggcttagcatcccataacgaaacacattaatatttctgcagaaaacaatatacgagtattcatacatctgttcaggttaggttttggctacccaatgagttttggtgttacattattttgttcagaaacactgggatctctgaagtgtggataagggcttgtaggtctgtgtaaggttttgctattattattgttgaatgtgcatctgatataactgccatgcagttgcttcttgaggacaactctgagcttttatgcccaaggccctcctggactcttggagttttctagcagggccttcctgcaccaagagctctgaataacctttgaaggctgacaggacactctcttcttctctctctacctaggtcctcaatttagtgatgtctccctgttcctctcagtgtggtaatagaggttggcaggggaggggtaggttgcaaatgcaatctccaggagccttccccagcctgaccctcaccccctcaaccccagctggtcccagtgggggaggggcacaggttgtgtggaagtgatgagtaagcccctcttctggtgaagctattgtgggttcaggcaatcgtctggcctgcacaggcaagataatggagtcaaaggaggcttatggcccctcagccgcccctgggcatgcacagatgtctctatggcacacactagcacttgcagaaaagcattggtgccaggtgcggtggctcatgcctgtaattccagcactttgggaggccaaggcgggtggatcacttgaggttaaaagttcgagaccagcctggtcaacatgcaaaaccccgtctctactaaaaatacaaaaattagccggatgtggtgacgggcacctgtaatcccaactactcgggaggctgaagcaggagaatcacttgaatctgggaggtggaggttgcagtgagccgagatcgcgccactgcactccagcctgggcgacagagtgagactctgtctcaaaaaaaagaaaagaaaagtgttggaggggaacgagaaagttcccccttaattctcagccagtatttactgagtgtgaccctgggctgggccccaggctaggtgctggggacacacagtgaggaaaacctggcccctctgagataaacccacaggccaggggcagctgccttctgacattgggggtatggggctggccctcaccctgaccatggtggcaggtgcccacccacccttcaaagcaagaggagggagggagaagtgcctgtatgttcaagagttactttacaaggacaaatgggtccatcaccttggttgacgtcagcaaagaagcatcagccaaagccttgaggtgaccccaaaagactggggtgcaggttagggggttgagacaggctcagcatggagagaggagggtaaagctcctgcagaggccccagctcccaaagatgaagctaccgcttgatgatgctgtctccagggccagagatcttcctctcatcccgcactatctgcagtcctctctggtgtgtgtggggcgcagtcattagacccatcttccaggtgagagatctctgcctcagggctcagaggacctcctcctggggtttcagatcagtcttccaggatggaggatgggaagcaggccatcaagagttctggtaagaaatgaggtttctagtcaggtacggtggctgacgcctgtaatccaagtactttgggaggccgaggcaggaggatcacttgaggtcaggagttccagaccagcctggccaacatggtgaaatcccatctctactcaaaatacaaaaattagccaggagtggtgaagtgcacctgtagtcccagctatttgggaggctgaggcagcagaatcgcttgaacccagaaggcggaggttgcagtcaactgagatcgcacactgcagtctagcctgggtgacagagggagactctgtctcaaaaaaaaaaaaaaagaaagaaagaaagaaatgaggtttccctgactgagtctgggaagctggcattcattcgttctttcactcattcattctggctgatcccgagctctgacagttcctatctgcatgaccctggcagctcacctcagccctgagcctaagattctactatgtaccaggcactcttcagtctacttaggatacagaaggagccaggtagtcatgacctccagcctcatgacgcagataatggggtgggggtaggggcaactagcttattctggaggcttcctgtaaaaaacaacgcttaagtggaggtggacagaatctccccatcacgctggggaaaggcagaaatggatttagcaaacttactgtgaaagtcacagcttaagccttagagcccctcacttgccaggggccttccaggggcctgggaggggccaagtaatgcacactcaggatcacatgctttagtagaatttgccaatgtaagatgttttaactgtaatttattaagactgctgcccctctcactccaacttccctctctgtcatacttccccttcttttgggtattgccccagtgcttctggcattttgggggatctagctaaggagaagttgtcacggaatactgacattgatgaaaataacaaaagtcaaaatacaccactacaaaaaggatgtaatagaaagcatcaattcaaaaaaattttaagattagtcatcaaggaaacataataagtccggaaatcttacagctccgatatgaaagaaacttgatagaggttcttccaaatttgacaacaatcctagaattttatgaccttccagtagtccccccttatcctcgagggatacatttcaagaccctcagtgggtgcctgaaaccgtggatagtacggaatcctatttagactatgttttttttgatccaatagccaagacaactactaagttgacgaatgggcaggtagtgaagatgctggacaaaggggcaattcacacccctggtgggacagggtggggtagagtggggcagcaccaaatttcattacgctactcggaacagcatgcaatgtagaacttaatgaattgttgatttctggaatttttcatttaatattgtcagactgtggttgtccatgggcaactgaaacctcaggaagcaaaaccttgcagaagagggggctactgtaccagtaataagttgcaaagctgaaagaaactttatcgaccataagaaatttggggccaggcacagtggctcatgcctgtaatccccgtattttgggaggccaaggtgggagggtggcttgaggccaggagttcaagaccaatctgggcaacatagtgagactccatctctacaaaatcttaaagtattagttgcatgtggagacacatgcctgtagtcctgattacttgggaggctgagacggggagatcctttgagcccaagagtttgaggctgcagtgtacaaagatcagacaactgcatgcctgcctgggcaatggagcaagaccctgccttaaaaaaaaaaaaaatgggggccgggcacggtggctcacacctgtaatcccagcactttgagaggccaaggtgggtgaatcatttgagaccaggagtttgagaccagcttggccaacatggtgaaaccctatctctactaaaattacaaaaattcgccaggcgtgcctgtagtcctagctactcaggaggctgaggcaggagaatcgcttgaacccaggaggtggaggttgcagtgagcctagattgcaccactacactccagcctgggcgacagagcaagactctgtctcaaaaaaaaaaaaaaaaaagaaaaaaaaattagtcaactgtgctagagaaaagattaaagtatcttcttattctctctaaagaaaatgacattacaaaatcaatgtcacatgaagaggttaacgtaaaagtatacaaacacaatgtaggaatgaaataattatagatatgtatcatattgatgaaaatatgaatgtaaatgtaaattttaatttatgtaattatgaacaaaaatgtaatgctattatgtaaataaatatatttattatgttacatgtaacttaacatgtttaataacttattatgttatgaactgttgctgactatgtggccacaacaggggagggaatcttgggacccttattcagagagatcaagaccaaataaaggacctaataagtcatttccttcaacctgtcaccagtgcaggaatcctcttcctgatgacagctgtccactgagcctcggctctgtacatttcctgggatgaggaattcacccctcctccaaatcctgtactatcttgggtcaaaactctggttgtgggaagttctttagtcaagctgatcactagctgtcggtggtttccccttgggtcctcatcttccccagcacccccagaaatcatgggctgctgcttcccattttattatagctctgcagtgctacaatgcagctctagtatcttgccctggcctgggataacctgcccttcttcaaagtttccttttatgtcttgacttccaaagtcttcctcatccatgatcgcagagattgatcagccactcatacatatatgaggacgacaatgatgatgatgataatgagaacagctagccagcactgagtgcttactgtgtactgggctccgtgctgggtgctgtatgagcacctgctgttggtctcatgcacacctatttatgttggttttgagtaacttgtgcaggtatacctttgatttaaaattttggtttctatttagactacgataggaatttttgttttgtttagccttctctcctaagcttaatgaaaccacatattcagaaagaaaggacacatttaattaaaacatttcaaagacacacagcttaaaagagtgattaccctagacctcttacaaacaaatatgcccctcctccaaaactcttcttaatgtaaatttcagagaggaaaagccaaaaacaaaaacaaaatcgagaatgtgtgttaatttatctggctaaaacctgataaaaagattttcttggccgggcgcggtggctcacgcctgtaatcccagcactttgggaggccgaggcgagcggatcacgaggtcaggagatcgagaccatcccggctaaaacggtgaaaccccgtctctactaaaaatacaaaaaattagccgggcgtagtggcgggcgcctgtagtcccagctacttgggaggctgaggcaggagaatggcgtgaacccgggaggcggagcttgcagtgagccgagatcccgccactgcactccagcctgggcgacagagcgagactccgtctcaaaaaaaaaaaaaaaaaaaaaaaaaaaagattttcttaagagctctgtagttcaaagtcaacttaattaaaagcaggtattaagactataatttttaaaatagagcctttctgcttcttctattttggatcttgttttggggaattttttttcaggtgactgaaacccctcttttaattatatggtgagtccctctctctgttcgcttcctttcttgttggtgtgattttttgctgaaggaaaaaaaaaatgtaaaacttaagcagctttctggaaagcttaaatttattctctgtgctttgaaatgtaaatttcctaccttgtctaaaattcagtgaggtactcgcttcgcagcacatatactaaaactggaatgaaggccgggtgcagtgactcacgcctgtaattccagcactttgggagtctgaggcgggtggatcacctgaggtcaggagttcgagaccagcctggccaacatggtgaaaccccatccatactaaacataaaaaaattagctgggcgtggtggcacatgcctgtaatcctggctacttgggaggctgaggcaggggaattgcttgaatctgggaggtggacgttgcagtgagccaagactgcaccactgcactccagcctgggtgacagagagagactctgtctcaaaataaataaataaacaaataaataaataaaatgaaattggaatgatagagaaaagattagtagcatgtcacctgtgcaaggatgaaatgtaaattctgaagcgttccattaaaaaaaatatgttatttaataaaattaattaaggccaggtgtgatggctcacacctgtaatcccaacactgggaagctgaggtcaggaattcaagagcagcctggccaacacggtgaacctagtctctattgaaaatgcaaaaattagctgggcatggtggtacacgcctgtaagcccagctactttggaggctgaggcaggagaatagcttgaatccaggaggtgggaggctgcagtgagccgagattgtgccactgaactccagcttgggcaacagagcaagactctgtctcaaaaacaaacaaacaaaaaaatgaaaaaaaaataagtcacaaagggatcaaacttcattttggctactcctgctttggcgatggccacaaaagggaaaaagtttttcaaatttttttggtaactatgcctttagagttttgccaagctaaattaaactatgaatatttattgaagatctagatcatttccaaataagatataatgctaagacattaattactacatataagtttaagctcatatacttttggtttcttatttcagagaaacaaaagatatttaggggctgggtgtggtggctcatacctgtaatcccagcactttggaaagctgagataagaggactgcttgaggccaggagttacagaccagccagggcaacatagtgagaccttgtctctacaaaataaaaattttaaagttagccaggagtggtgttgcatgcttgttagtcctaactactcaagaggctgaggcaggaggatcgatcactcaagcctaggagtttgaggctgcagtgagctataatcacaccactatattccagcttgggcaacagagcaagaccctgtctcaaaaaaaaaaaaaaaagagatattaagatccgctagtaaaagtatcctattccacactgaaaaattgttccattagaaagcctgtgtttctaaatattataaaatgtgtattaatcaattgttagtacatagtgacaaaattacttctggctgggcggtggctcacacctgtaatcctagcactctgggaggctgaggtgggcagatcacctgaggttaggagtttgagaccagactggccaacatggtgaaaccctgtctctactaaaaatacaaaaaattagccaggcgtggtggtgtgtgcctgtagtcccagctacttgggaggctgaggcagaagaatcacttgaacctgggaggtggaggttgcagtgagctgagatcgcgccactgcactgcagcctgggtgacagagtgagactctaaaaaaaaaaaaaaaattacttcttagattttcagtataaattaagattactaagatttaaaattctgactaatatatggtaactaacactagagaccagaaggaagacaattctgtattcagaatatgtaaggaaagtaagacatctttttaggaaggaagattataagaaagacataagcatgtggtttttgttaaagagaaagtggttttgcctagtttagaggttatttaaaggctgtatgaaattgggataaaagaaggaaagaataaaatagattaactgaatggatatagaaagttgggaaaagaaagaggaatggaaaaattgtaagaagttataaaaggtttatagaaatattatctcgtgtggtcaaagctgattgagattagatgatttataaggttttattaaaattaggctttatatttataatgcattgatgcaaaagtagaatcatttttctattttgaactagatagtcacatagttttttttttgttcttttttttttttttttttgagatggagtctcgttctgtcacctaggctggagtgcagtggcgtgatctcggctcactgtgacctccacctcctggattcaagtgattctcctgcctcagcctcctgagtggctgggattattggcatgcgcctccatgccaggctaatttttgtattttgagtagagaaaaggttttgccatgttaaccaggctagtcttgaactcctgatctcagggtgatccgcctgccttggccttccaaagtgctgggattgcaagcgggagccaccgcaccctgcctcatatagtattaataagagatagcaaaagatttttttgtttaccttttgagtaaactgctgctaaaaaaaaaaaaaaggagaaaagaaacgggggagagggagagacattctgttggtctcaagttgtctttttcaggtcttttgtgtcaggcctctgagcccaagctaagccgtcatatcccctgtgacctgcatgtatacatccagatggcctgaagcaactgaagatccacaaaagaagtgaaaatagccttaactgatgacctttcaccattgtgatttgtttctgccccaccctaactgatcaatgtactttataatctccccccacttaagaaagttctttgtaatctcccccacccttaagaaagttctttgtaattctccccacccttgagaatgtactttgtgagatccacccgctgcccacaaaacattgctcctaactccactgcctatcccaaaacctgtaagaactaatgataatcccaccaccctttgctgactctcttttcggactcagcccgcctgcatccaggtgaaataaacagccttgttgctcacacaaagcctgtttggtggtctcttcacacagatgcgtgtgacatttggtgctgaagacccgggtcagagggactccttcgggagaccagtcccctgtcctcaccctcactccgtgaagagatccacttacgacctcgggtcctcagatcaaccagcccaaggaacatctcaccaatttcaaattgggtaagtggtcttttcactctcttctccagcctctcttgctacccttcaatctctctgtccttccaattccagttctttttcctctccagtagagacaaaggagacacattttatccgtgaacccaaaactccagggccggtcacagactcaggaagacagtcttcccttgccatttaatcactgcggggacgcctgcctgattattcacccacattccattggtgtccgatcaccgcagggacgcctgctttggtcattcacccacattcccttggtggcaagtcaattgcggggacgcctgctttggctgctcacccacattgcagcccagggctgctccccacccccttctccatatctctacccttctctttaaacttgcctccttcactatgggcaaacttccaccctccattcctccttcttctcccttagcctatgttctcaagaacttaaaacctcttcaactctcacctgacctaaaatctaagcatcttattttcttctgcaacaccacttggccccaatacaaactaacaatggttctaaatggccagaaaatggcacttttcatttctccgtcctacaagacctagataatttttgttgaaaaatgggcaaatggtctgaggtgtcttacgtccaggcatttttcacacttcgttccctccctagtctctgttcccaatgcgactcgtcccaaatcctccttctttccctcccacctgtcccttcagtcccaaccccaagcgtcgctgagtcttgtgaatcttccttttctactgaaccatctgacgtctcaccttcttcccagactgctcctcctcagctcgctccccaccaggctgaatcagcctccaactcttcttcagcctctgctcccacatcctataacccttctattacccgccctccccacacccagtctggttttcagtttcgttctgcggctagctctcccccacctgcccaacaatttcctcttagagaggtggctggagctgaaggcatagtcagggtacatgtgcctttttctctatcagacctttcccaaatcagccagcatttaggctctttctcatcagaccccactaaatatatacaggaatcccgatatctaactctgtcctacagtttaacctggagtgactgaaatgtcatcctgacttctaccctctccccagatgaacgggaaagagttttttctctagcccaatctcacgctgataaccgccggcttcatgaacctgacctccaggaaggcagtagagcagttccccgagaggacccccaatggaactatcaggcagattccccaggtatggctaggcgagattacatggtttcctgcctagttgaagggcttaaaaaggcagcttacaaagctgttaattatgacaaacttagagaaactacccaaggtaaagacgaaaacccagctcagttcatggcccgctcggcagcaacccttacacactttaccgccctagacccagaggggccagaaggccgccttattcttaatatgcattttatcacccagctcctgacattagaaaaaagctttaaaaattggaatccggccctcaaaccccacaacacgaattaatcaacctccccttcaaagtgtacaataatacagaggaggtagccaggcagcaacgcatttctgagttacagctgctcgcctccgctgtaagacagcccacaaccacgtctccagcatacaagaacttcagaacatccaagccacagctcccaggggctccttcaaaacatcctcgtggaccttgcttcaaatgctaaaagcctggccactgggcctcagaatgcccgcagcccgggattcctcctaagccgtgccctgtctgtgcgggcccccgctggaggtcggactgtccgactcacatcactgccactcctaaagcccctggagcccaaaccctatgttccttggccgactccttcccagatctcctcggcttagcagctgaagactgacgtagcccgatcgcctcagaagcctcctggaccatcacagacgctgagcttcgggtaactcttaaagtggagggtaagtccatcccgtttaatcgatatgggggctacccactccacattatcttcttttcaagggcctgtttccctcgcccccataactgttgtgggtattgatggccaagcttcaaaaccccttaaaactcccccactctggtgccaacttggacaacgttcttttatgcactctttttcagttatccccacctgcccagcttccttattaggctgagacattttaaccaaattatctgcttccctgattattcctgtactacagccacatctcattgcccccttcttcccaacccaaagcctcctttgggtcttcctctcatatcccccgaccttaacccacaaatatgggacacctccactccctccctggcaaccaatcacatgcccattactatcccattaaaacctaatcacgcttaccccactcaatgccagtatcacatcccacaacaggctttaaggggattaaatcctgttatcacttgcctgctacagcatgggcttctaaaacctataaactctccttacaattctcccattttacctgttcaaaaaccggacaagtcttacaggttagttcaggatctgtgccttatcaaccaaattgttttgcctatccaccctgtggtgcccaacccgtacgctcttttgtcctcaatatcttcctccacaactcactattccattcttgatctttaaaatgctttttttcactattctcctacaccccttgtcccagcctctctttgcttttacctggaccgatcctgacacccatcagtcccagcagcttacctgggctgtactgccgcaaggcttcagggccagccctcattacttcagccaagctctttcttatgatttactttctttccacccctctgcttcttgccttattcaatatattgatgaccttctactttgtagcccctcctttgaatcttctcaacaagacaccctcctgctccttcaacatttattctccaagggatattgggtatccctgtccaaagctcaaatttcttctccatccattacctacctcagcataattcttcataacaacacatgcgctctccctgcggatcgtgtccgactgatctctcaaaccccaggcccttctacaaaacaacaactcctttacttcctgggcgtggttggatacttttgtctttggatacctggttttgccatcctaacaaaaccattgtataaactcacaaaaggaaacctagctgactccatagattctcaatcctttccccactcctctttctgttccttgaagacagttttagagactgctcccacactagctctccctggctcatctcaacccttttcattacacgcagccgaagtgtagggctgtgcagttggaattcgtacacaaggactgggaccgcaccctataggctttttgtccaaacaacttgaccttactgttttaggctggctatcatgtctccatgcggtggccgctgctgccctaatacttttggaggccctcaaaatcacaaactatgctcaactcactctctacagttcttataacttccaaaatctattttcttcctcacacctgacacatatactgtctgctccccggctccttcagctgtactcactctttgttgagtctcccacagttaccattgttcctggcccggacttcaatccagcctcccacattattcctgataccacacgtgacccccatgactgtatctctatgatacacctgacattcactctatttccccacatttccttctttcctgttcctcaccctgatcacacctggtatattgatggcagttccactaggcctaatcgccacacaccagcaaaggcaggctatgctatagtatcttccacatctatcattgaggctaccactctgcccacctccactacctctcagcaagctgaactcattgccttaactcgagccctcactcttgcaaaggaactacgcactacgcatcaatatttatactgactctaaatatgccttccatatcctgcaccaccatggtgttaaatgggctgaaagaggtttcctcactacgcaagggtcctccatcattattgcctctttaataaaaactcttctcaaggccgctttacttccaaaggaaactggagtcatacactgcaagggccaccaaaaggcatcagatcccatcgttcagggcaacgcttatgctgataaggtagctaaagaaagagctagcattccaacttctgtccctcacagacagtttttctcctcctcatgggtcactcccacctactctcctgctgaaacttccacctatcaatatcttcccacacaaggcaaatggttcttggaccaagaaaaatatctccttccagcctcacaggcccattctattctgtcatcatttcataacctcttccatgtaggttacaagccgctagcccgactcttagaacctctcatttcctttccatcatggaaatctatcctcaaggaaatcacttctcagtgttccatctgctattctactactcctcagggattgttcaggccccctcccttccctacacatccagcttggggatttgcccctgcccaggactggcaaattgactttactcacatgtcccgagtcaggaaactaaaatacctcttggtctaggtagacactttcactggatgggtagaggcctttcccacagggtctgagaaggccatcatggtcatttcttcccttctgtcagacataattcctcagtttggccttcccacctctatacagtctgataacggattggcctttattagtcaaatcacccaagccgtttctcaggctcttggtattcagtagaaacttcataccccttaccgtcctcaatcttcaggaaagatggaacggactaatggtcttttcaagacacacctcaccaagctcagcctccaacttaaaaaggaggactctgtcaaggatacagcccaaaaactcaacaaccaagcaagtaattacgctgaacagccttgggcactctctaattggatgtcctgggtcctcccacttcttagtcctttaatacctatttctctccttttattcagaccttgtgtctttcatttagtttctcaattcacacaaaaccgcatccaggccatcaccaataattctgtatgacaaatgctccttctaacaaccccacaataccaccccttaccccaaaatctttcttcagttgaatctctcccactgtaggttcccatgctgccccaatcccactcgaagcagccctgagaaacattgcccattatctctccataccagccccaaaatttttcgccactccaacacttcaccactattttgttttgcttttcttattaatataagaagacaggaatgtcaggcctctgagcccaagctaagccatcatatcccctgtgacctgcctgtatacatccagatggcctgaagcaactgaagatccacaaaagaagtgaaaatagccttaactgatgactttccaccattgtgatttgtttctgccccaccctaactgatcaatgtattttataatctcccccacccttaagaaggttctttgtaaccccccccccgacccttaagaaggttctttgtaattctccccacccttgagaatgtactttgtgagatccaacccctgcctgcaaaacattgctcctaactccaccgcctatcccaaaacctataagaactaataataaacccaccaccctttgctgactctcttttcggactcagcccgcctgcacccaggtgaaataaacagctttgttgctcacacaaagcctgtttggtggtctcttcacacagacgcacgtgacattttgattgtttggaaaattcagtctcctctctatgaaagagtaaaagtttgctttttgaaatatttgaatcatcactttggctagatgaatgactacaattttaaactcactttgccaacacactgacattggcagagtgcaaagatggcaagaggctgggtccatggtgacactgttagggaaacaggagcataacagagtcagggtgacaccattttaaaatcaattgtggctgggcacagtggctcatgcctgtaatcccagcactttgggaggctgaggtgggcggatcacctgaggtcaggagttcaaagccagcctggccaacatggagaaaccccatctctattaaaagtacaacaattagttgggcatgatggtgggcacctgtaatcccagctacttgagaggctgaggcaggagaattgcttgagcccgggaggcagagtttgcagtgagctgagatcgtgtcactgcactccagcttgggtgacagtgtgacactctgtctcaaaaaataaaataaaataataaaataataaaatcaactgcatcttcaaactagcaaggcacattccttggcagtcacaactcatggccatgatatgttttgggtgaaggaagcgatttagtaatgcctgcaagggcaaactcctatggtggcagggtgtccagatatcctaatagcacataacaatatctgcttttgagataggtaaagtcatgctttgaagtatttcctcactaaaataccaaggataattttatttaaatcaacaaagcactaaattttcttttttcttttttgagatgctcactctgtcgcccaggctggagtgcagtggcacgatctcggctcactgcaagctccacctcctgggttcacgccattctcctgcttcagcctcccaagtagctgggactataggcgcctgacaccatgcctggctaattttttgtatttttagtagagacggggtttcaccatgttagccaggatggtcttgatctcctgacctcgtgatccacccgccttggcctcccaaagtgctgggattacaggtgtgagccaccacacccggcctaaattttctttaaaaaaaaaaaattattgtatttatggctgggcactgtggctcatgcctgtaattttagcactttgggagactgaggcaggcggatcacttgaggccaggagtttgagaccagcctgggcaacatggcaaaatcccatccctaataaaaatacaaaaaaaaattagctgagcatggtggcacatgcctgtagtcccagctacttgggaggctgaggtgggaggatcacttgaacccgggaggcagaggttgcagtgagccaaggtcgtgccactactctccagcctgcacaacagaaaggactccatctccaaaaaaaaaaaaaaaaaaagtatttatttatttttcatttattccaggcagaagaaacagcaaatgcataggtcctgaggcaggcatgcatttggcatgttggaaaacatgtggcactggccagaccaagcaaggccttggagaacatgaagagcagtctggcttttgctccagttgccacagaagtcactggaagaggcctcctctgagataagacactaagaaagcagtgtcaggccagttagacaggtctggacttgtcttctggagtcaaatgcaggcggcagacatttaaatggccagtcacagagagggtgatgggggccatgatgggtgacccacagggccgtgagagcacagaggagggaccctgccccatcctgagggcccaagggtccttcccaggggaagagagagctcagctgagacctgaaggctgcagcagagttagccagcttgaaagagaacgacaagggatgggatgggaagtggattccaggcagaggaagaagcaactgcaaacgcctgagaagagaaagcctggagcatttgggggaccagaagggggttaatgtggctggattgtagatgcaaacaggggttggcctggggggcaggcggcagcggctaggagggctctgcttttctcacttgatatactgtgaacatttttctatgtcagaaaggatccttctgctataggatttttaagggctgagcattacgtcgtggaataactggttctccagtgtcagacatttaggttctttctagtttttccctcttagaaacaatgctatgttgaacatctttgtctgtgcatctttgtgcacacgtattattatttctgtgcggtaaagttgggaagtctcggaggctacttggtggacaggattgagagctgccttggagaggcctgagtcagatctgtttgccagatcagcctccactgggtttctactggaggggccatacacagggagatgcagggagaaggcctgagggagagatagagagccctgattgtgagctgtggctgcccaggccagataatggcaggggagagaggaggccccgatcctgggcccctgtctgtgctgtcggcctggtgcgttagctcctggtgccttctaaagaggcaacaaaagtacttcaaattgagcatgagcttgggttcaaatcacacctctaccgctaaaaaactaagtgccgttgggccagttacttagtcattctgaatctcagcgtccttatctgtaaaatggggaaaataagccaatagggttattgtgaaagatacatgagattaatgagtcttggcgatagtccctgctcccagtaaatgacggcgtgcatttttattgtcatcttgggtctccatcctttttaaaaaaatacttgattataacagctttattgagataaaattcacatgccatacaattcacccatttaaagtgtacaattcaggcagggtgtggtggctcatgcctgtaatcctggcactttgggaggccgaggcgggcagatcacttgaggtcaggagttcgagaccagcctggccaacatggtgaaaccccatctctacaaaaaatacacaaattagctgggcatggtggtgggcgcctgtaatcccagctactcgggagactgcggcaggaggatcgcttgaacccgggagatggaggttgcagtgagccaaggtcatgccactacactctagcctgggcaacagagcaagactctgtctcaaaaacaacaacaacagataaagtgtacaattcaatagttttttatatatttgtcacaatcaattttggcactttttcattatcccccacagaaaccctgtacctatcagcagtcagtcctgcagccgacccccctctggccccaggtaactgccaattactttctgtctctatggatttgctctttctagatgtttcatagaaaagaagtcatgcaacatggggtctttttttttttcttttgagacagggtctccttctcttgcccaggctggagtgcaacagtgcaatcacagctcactgcagcctcgaactccagggctcacatgaccctccctgctcagcctcccaagtagctgggaccacagtgcaccgccatgcccagcaaatttttaaaaaattgtttgtagagatgggttctccctatgttgcccaggctagtctagaactcctgggctcaagtgatcctcccaccctggcctcccaaagtgctgggattacaggcatgagccagtgcgtccaggcctgtggtcttttatgactggctttgttcacttttttcatccctgtcagcaatgtatgagagttctgatttctctgattccttaccaacacttattattgtttgtcttttttattgtagccatcctcgtgggggtgtgtagtgggatctcattgtggctttgatttgcatggccttgacggttaatgtttctggtttttttcagtggaatcccctttataaattctgggacaccctattcccagtgtggaaacactaacctgttccaaagaaagaaaaaaaattctagatggaaaaagatgttcattactgcgacataacatttcttaatacaagtgactcgtctatagcagtaggtagttcctaatttttttttttttttgagacagagtcttactttgtcacaggctggagtgcagtggcatgatctcagctcactgcaacctctgcctcccgggttcaagtgattctcctccctcagcctcccaagtagctgggactacaggaacataccaccactcccggctaatttttgtatttttagtagagatggggtttcacaatgtggaaacactaggccacattgtgaaatgtggccaggatggcctccatctcctgacctcatgatctgcccacctcggcctcccaaagtgctgggattacaggcgtgagccaccgcgcctggcctattatctttaataattataaatactgggctgggcgtggtggctcatgcctgtaatctcagcactttgggaagccaaggtgggcagatcactggaggtcaggagttcaagaccagcctggccaacatggtgaaaactcatctctattaaaaatacaaaaattaccctgtcatggtggtgcatgcctgtaatcccagctactcagaaggcttaggcaggacaatcgcttaaacctgggaggcggaggttgcagtgagccgagattgagccactgcactccggcccaggcgagagagtcagactccatctcaaaataataataataattataataactataaagaccagctatcatatggaaaatgtccctgatgtgtgaacaaatgcaggatggaaaaatactcagtgtagtcattttagctaatatatatttgttaaaacatccaaatatttttttcgagctcggcgctgtgtgccaagctccatgctggctcatggacaaagtcaggaaaagaacaagcaaaaatgaaattccttcttgtgtcgggagtggtggggttttgggggacaggtatctccccttccccatgttttcttctcaaacttcctccactgttgttatattacctttgcagtgataaaaccaagagaacagaagaaatacttctggacctaaggatgaaagaatgatgggagaaacatttcttgagccagtccctttctgcgttcttattttgtggaatccgcacacatccccgagaagcttaataaaaagggctactatcatgacacttactgtgtgccttgccggttccacctgttaggtgccattgttgtccccattttacagatgaggaaactgaggcggggcaaggagatgcccttctgcttggtggtctatccttcagcattacccacacacatgcagagctacatataagctcacgttcacactcggattcacgtctgcacccatgggcacatggaggatcgcacaagccacactcagacacacatgtgtgctcacacacagggctgcccatgtccacaggtatgtgcatggggacacgcatgtatatatgtgcatattcccatatgcacacagcacaggtcaaacacttttggacacacatctgcctgagaatgggaaaaggggtgcaagataaaggggcaaagtctggcttttgcctcctccctgcacctgctaccagctgtgtgcaggactgggtggggcagaaataggtggctctgagctcagagggcagaggtggccttgcactagaaatccacctgccaaacttccaaatgggctacagcgactaaggggcctcacctgctgggcaaatcccccagctggagggtgtgctccagatcctccaggggtccccagggggttgagaagatgaggggcacacccagcagcccctaagggaggaagcgtggccatactggctaagggggcgcactcttcttgcaggccgcctgatcagatgcctgtaaaataagacagctttacaaagagggtgtcggaatgtgaggaggcagagggacaggcatgagtagaaagaccttcctcaggacctgaagtccaatgatcctggtcctgcgtcccactagctaggtgatattgaacaagtcacataacctctttgaacctcaatttcctcatttgtaaactttgcacaaatcatttctttgactgctaaacaagtatgttttgaggaccaacgacatgccaggtacggtgctgggcactgggaaaacagcagcaagcaacacagacatgggcttgccgtgtagagcctgcagaattagggaaaggataaatggaaacatctcacacatagtaagtgctcagttacgttcctcctggtctctcttttctaccattgtaaaggcgatgcaataacatagaaagttgggagaatggggtggcggttgctgaggggggaactctgtcatccagaatcccaccaccccaacacaatgactagcttcatttttgccaatttcatcagctcatgcaggggttgacctgctgtagggcactcaaaatattcaaaccaattaatgcattgcatttgtgatcagaagaaaaaagctaattacaatgtaacagatttacctgatgcaaagcaacgcaagcatggccatccctctgcatatatggaagcttttccttttgggggaaacagcaatatttccattttacggaaaaagaaatggaggcacagagaggtcaaggcacttgcccaaggtcacacagacagaaatgcgaagagcagctccagaggccagaactcctgcccatcctgtccaggactgtgggatgcatccagggacggacactggggctgtgggctggatgacttggctgcctttgcattgattggagctgtttagggaacctaccccagccactagcatccagtcctagagacacagaaaattcactggccagcctcacttttgagcccagaaaccccttacccttcctcctgcctcttgagaggccagtgttaggtgttagccggggtgcaaagctctggaaggcaggtttctgctttctgctgccctccagtgggcaaagaaagcaaacctctggatccatctggaagcaggtagcaggtgttgcccaagtcagctgcggctaatagtaataataatggctgccgctcaatgagcacttaccacgtgcagacgtttttacacctaatctaatgtaacctaacccctttaagcaatttaattaacatttaattcctctctcaaggtaggaatcacttcctatatacccatttacatacataatctgagacttagaaaaatgacttcccaaagtcacaaagctggtcagtggcagagccgagagtgcaagtccttggagatcagaggaggaagagaccatgatcctggaccaggagacagccctgcattcttgggcacagaggtgaatttactgtgaggctggtgacgcatcagggctcctgacttgcatgtcctctcccagggccatggaggaactttccaacgcattcgcatgggcatatgtttcacatttgcaaaactaacacatttcagttgcaattggctgagaccactatctctctccactgcctagaataatgtcttcacatagtaggtaataaatatgtgctaataaatccattttgtgtttaataaatcatgttgaatgaatgggtagagaaatgaaggaaggaaggaagtggcatttagttcaatcttgaaggaagggcaggatttgagagagcgttcctcatgtagcctagtgggcccctccacacacagaccatccaaggccatgagtggccttgaatgccagggtgaggaatctggccttaggtggtaggcactggggagccatggaaggttgcagagcagaggaaggatatgagtgtaattgtcaattaggcaagagttgaatgtcaaataagaggacagggccctacagcggggggccagagtggctcagataaaactcccctcatccagcaccacacagagagctggtgctcagccagtgtgatcacagaagcctctgctggggtgtctataagctccctggaagaagatatccaaatgctttgcatgtgtggctttgtgtatgtgtgtgtgtgggggggggaggggaggtgctgagtgtggatttgctcagcactctagtgtgcccagcccaacgtgggggaaaggtcaaggccctgtctggcttaggcagggagttctcagcattgcagtatgactgagcctctggctggaaagtaagggagccaagagaaaacaggtttagaagttggctaggcagaagtggacctatgaaattccagctgcaccagctgcttcttttgctaagctcccgtcatcctttctctctctccactgggtctttctgaatgtcaagaatcccagccactgtttagttagcacttgttttttgccacactctgtgaagcaccttcaagcccgatcaccggattattcctccaacaacgccgagagtgagaagaatggctattatttcgattttataggtgaggaagtagaaagcccagagaggtgaagttgcttacctgaggtcacataggagtcaatggtatacgtgagatcaaacccagactccagaggcagcccccctcagtcgccagccgtcctgcctcctctcctggtctaagctggggaggaaaaacccatcttggccagcagggggcggtgtgccctcaaggataagccctgcttcccagaactcagacagaatttgccagcaagacaacagcacgattctgaaatatctggctttgagccctcatttagtcccaactctggtggggcctggagaacggggagaggggtgagagaagtataaaatagccctcaaattggtgagccaatggttcacagaaaggaaagcgcagcggcattttaacatataaaaagattctcattttcactcctaggaagagaaacgtgttaaacccacaccacctgagcaggcactgttttgctatcaaactggcaaacttatgcaggtggggatatggagacacactccttcttacattgttggtgggattaaaacttggttttggccaggtgcgatagctcacacctgtaatcccagcactttgggaggccgaggagggcggatcacctgaggtcgggagttcaagaccagcctggccaatatggcgaaaccctgtctctactaaaaatacaaacattagctgggtgtggtggcacacgccagtagtcccagctactcgggaggctgaggcaggagaatcacttgaacccaggaggcggagcttgcagtgagctgagatctcgccattgcactccatcctgggcaacagagtgagactccatctccaaacaaaccaaaaaaaaaaaaaaaaaaaaaccagaaaagaaaacttggtttaacacctatagaagctaatctggtaacatctatcaaaattaaaaatgcacatatctaacaggtatgcatgatacattcatcaaaagacttgaactagacctgcatgatctgatgtggagccacccaccacatgtggctgctgagtccttgaaatatggctgatccaagcctggctgacatggcaaaaccctgtctctactaaaaatacaaaaatcagccaggcgtggtggcacgtacctgtagttccagctacttgggaggctgaggcacaacaattgcttgaacccaggggcggaggctgcagtgagccaagatcgtgctactgcactccggcctgagcagcagagcgagacagtctcagaaaaaagaaagaaatatggctggtcaaattgagatgtgctgcaagtgtgaaatatatatgggattttgtatactaacaaaaatgcaaaatgactccttaataacttgctaatattgatgatgtgtcgcaataatattttggatagattggattaagtaatttttatttttgttttttatttttttgagacggagtctcactatgtcgcccaggctggagtgcagtggcatgatcttggctcactgcaacctctgcctcccggattcaagtgactctcctgcctcagcctcctgagcagctgggactacaggcacctgctaccacccgtagttaattttgttttgtatgtttagtagagatggggtttcaccatgttggccaggctggtctcaaactcctgacctcaagtgatctgcccacctcagcctcccaaaatgctgggattacaagcatgagccactgtacctggcctgggttaagtaatttttaaaattacttttacctatttctttttcttttttgaatgtggctgctagaaatatacatggcttgcattgtggatcatattatatatttttacctttttattgtggtaagatatgcataacatttaccatttggaccatttttaagggtccagaagttcagctgtgttaagtacattcccattgttgcgcaaccatcaccatcatctacccccagagcgttttcatcttcccaaactgacactctgcctctataaaacaacaactccgcttgctcctctcctcccagcccctggcagccactattctactttctgtctctgtgaactggactattctaggttgcctcatacgggagaaatcatatacaatttgtccttggttgctggcttatttcactcagtatagtgtcttcaaggttcacgcatgttgtagcatatgtcagaccttccttccttttttaagactgaataatgttccattgtaaggatataccacattttgtttatccattcattcactgatgggcatttcggttgtttccacttttggctatggtgaatagtgctgctgtgaacattttggtacaaatatctgtttgactcatattttcagttcttctgtgtctatcatattttattggacaggactatgccagtgatctccatagccacataatttgaaatatccctaaaccaggaactacccaaatgctcatcgacagcagaacggataaattgtggtatcttcatacaatgcaatactccagtgagaatgaaaatgaatgaacaactacacacagcagtgtagatggaacttgcacacatatgtgtcgagcaaaagaagccacacgcaaaataatacatattgtgtgattccactcacaaaaagttcacaagaggcaaaactaatttatgatgttaaagtcaggatgatggctgctctttgggggccatctgggggcttctctggggctgacaatgttctggacaccatcttcaggagcgtggtcactccgtgaaaattcatcaagctaagcacttgggatttgtgtgcaactttgtgtataagttagacttccataagaaattccaaaagatgctttgatccagcaattccactcttaggaattaaacgacagatatattttcatatgtgtgaaatgaggtgtgtacaagattatccactgccgtttttatcagcaaaagattggaaacatgccatctcacacctactaggatgactactatttttaaaaaatgaaaataagtgttggtgaggatgtgaagaaattggaaccattgtgccctgttggtaggaatgtaaaatggtataacagccacggaaaactgtacagcagttcctcgaaaaatgtaaaataaaattaccttatgatccagtcattctgcttgtgggtgtgtgcccaaaataactgaaaagcagggtcttgaacagatatgtgtacacccgtgatcatagcagcactattcacaatagtcaaaggtggaagcaatccaagtatccaacaatggacgaatgaataaacaaagtgtggtctatatgtaaatggaatattattcagccttaaggaggaaggaaattctgatagatgctacagcgtggatgacccttgaggacactatgctaaatgagatgagccagacaagaaggcacaaatactgtattattccacttagacaaagtatctgtctaaagtaggctggatgcggtggcttacgcctataatcccagcactttgagaggccaaggtgggcagaccacctgaggtcaggagtttgagaccagcctggccaacatggtgaaaccccatcttaactaaaaatacaaaagttagccaggcgtggtggtatgtgcttataatcccagctactggggaggctgaggcaggagaatcgcttgaacccgggaggcggaggttgcagtgagccgagatcgcgccactgcactccagcctaggcgacagagtgagatccgtctcaaaaaaaaaaaaaaaaaaagtagcccaattcatagggacagaaagtagaatggcaattccaggagctgggaggagggggaataggatgttagtgtttaatgggtacagagtttcagttttgcaaggtaacattttggagaggtttggtggtgatggttgcagaacaatgtgactatatttaatgccacaaaactgtacacttcaaatgattaattagctaatttttggtttttttttttttgagatgaagtctcgctgtgtcacccaggctggagtgtagtgacgtgatctcgactcactgcaagctccacctcctgggttcatgccattctcctgcctcggcctccctaatacctgggactacaggcacctgccacaacgcccagctaattttttgtatttttagtagagacggagtttcaccgtgttagccaggatggtctcgacctcctgacctcgtgatccacctgcctcggcctcccaaagtgctgggattacaggcgtgagccactgtgcccttcctaattagctaaattttatgttatgtatattttgctgcaattaaaatttttcaagtgaggtatctataaggaaaggtgagaaaatatgtaagatacaaagataataaaatccagagcaagaacagtatataagtcctg

SEQ ID NO: 5 - DNA, 13567 bp, Homo sapiens
ctgccccaccccgcgcggcccgcgccctgcgcggctctccggccccggcgcgccccggaggaacccggccgccgcttccctggggacggccgagcctgcccccgtcggcgcctccccaaaaagaggcccccccgcagtggctcccgaatgtcgggctcgccagcctcggcttcctacatggaaggtccgcgggggcaaaaaacgaaaggcgttcggctgggctgttggaagaaggaaaaagcctctttcccccttgctaagcaacttaatttgggggtggggagaagcaggcaattaaaaaaaaaaaagcaagcgatttatttttttcctctatatccttagtaaccggatctcctcgaattccgcgcacacgaagactcaggggagggggccgagtggacttcaccccgcatgagacgtctggcaaaataagaaggctctcgcaaaacctaacaaccaaatatgcaaagccccaaatgaaaaccaccacctcctcgaacctcagaggtctgggggcgtccggctggaactggggtttaaaaaaagaaaatgtttacaaagtataacaagatgtttgatgggtggaaaaatgtatccacgagttacatccccccgtttccttgcaaagccccgctggtcttcctctccttttcttctgccaaaaaaaaaaaaaaaaatcgtgtatttttttaatccacagaaagctttggctagaccgcttcaatcctgcgcatctgggtggtttaggggagtctctggtctttccccctgcgctcctgggggcccaggtcctcggcggggacttcctcgaggctggcgcgggcgcaggggcagaagatgctgcggcggcggctgagcccggcggggctgacagcgcgggggagggtggcgcggcggcggcggagggccccagacgggtcgcgcgttctcgccccccccgggcacaagctgcttgctagtgcaggggccgccgatgtcccttcccctggccgcggctggccgccgaggctccccgcatgggctgctcgcctcgacccagctgcggcggcaggaggccccggtgtcctctcggcgcctcctcctccgagactctcctcgtcgcgcccgggagcctccttgtccccggtccgccctctcctggcgctccggtccttctgccgccgccaggggctcgccgcgccgcactcaggggctcaggggccgggcgctcggcggctcggcgccgacggactggctctgtctcgggcagctctctcccgcgcggcgagcggaccgagcacggcgcccggctggctcggctggcgcggctcggggacaggatcttccgtgcgccgagcagcaagcgagtgtgcccggggctcaccgcctcccgcaaggcctcccgcccccgcccccttccctcccccttcctcccccttccctcccccgcccccagccgccgcagccgcgccgcctcctccccgcccccccgcaccccccctccggccctctgctcggctggttccactgcgcagtggcgcgcccggctccggcctcgtcacgtggccgtctagacaccctgtcgctttaaaaaaaaaaaaaaagcgattgtgtttcgcaaacaacagatcgggtttctaaaagctatttctccccccaaccccccgccaccgccaccccctcccgggtctgtagagggggtaccgatggaggggagagagataggtggggggcagagaagctcccagaatggattgagccccggccggagccatggagaaattggaaaagcagggagcaccgagcgggcttcgccgcgagttttggagctgagcgagcgggtcggtggcccgatttcgacccggctgggtttcgcggtggccatctcgcgcgcgctcgccctagcgcttcattcattggttttgttttaaaggccctggcggtggatcccttggccgcgcccgagggcaaggggaggagagcgctgtctcggtttaaaagacatttataccggactggaccgaggccctgggaagtgtgcgctgaggggaacagccgccgagggcggggaggcggcgtgaatatgacctcagcggcggccgcgcgctccctcccgccctctcagctccgggctccggtttctaggactgcctggagaagtgtgtcttgtgcacagctctggaatgcatttggccggctgacgagctgtgaggggcagcatcccggcgggagaaggggagcgggggtgggggctcgcctgcgcgccgcgggcaggtttcctcccgggcccggaagacctccgccacccgccaccctgcctcccggcgcgggaaggttacccagcgagcagacctgcctagggcattcatttgcatgcaggccctgtttctgggcctcgtagctttcaaggtgcttagagtcagagagtttattccttgaccccaggtcccgaagaaacatatacccaagctggcgggttactgcatagaaacgggcatggcattgctagggcataaacgcatttacagcgtgaaagctgatggctccgagaaacgtaatgatttaaatacacacacatcagtattgatgaggccactagttggcatggtgatctaacctcacttcatattcagtgaaatacgatttttttaaaaagccattgagaattgtgagatcaggccagcagtgaaactcgttgggggctttaaagaatctttttttctttctttctttctttttttttttttttttagagtctcactcttcacccgggctagagtccagtggctcgatttcggctcactgcagcctctgcctccccagatcaaacgattctcccacctcagcctccggagtagctgggactacaggcgcgcgccaccacatctggctaatttttgtattttttggtagtgacgcggtttaaccatgttggccaggctgatgtggaactcctgacctcaagtgatctacctgcctcagcctctcaaagtactgggagtacaggcgtgagccactgcacctggccttaaaataatctttagaaaaggtgaaatgtgcccaggtgcgatggctcacgcttgtaatcccagcactttgggaggctgaggcaggtggatcacctgaggtcaagagtttgagaccagcctggccaacatggtgaaacccgtctctactaaaaatacaaaaattagccaggcgggtggcgcgcgccagtaatcccagctgagacaggagaattgcttgaacccgggagacggaggttgcagtgagctgagatcgcgccactgcactccatcctgggcaacagagtgagactctgtctcaaaaaaagaaaagaaaaaaagaaaagtaaagatgaaatgtacatcttgccggctaaattatatgttcttaaaaggaaaaggcaggaatgaatcttagccgcctttagagctcaagtcctctccccctctagcaattaaaaagatttctaacatattagtacaatagtagatgcttaataaatatttagaaatcaacacttagggcttaaggggcatttggacccttcctccaccccaccaaaagtacctttggtaatataaattcaagaggaaatcagcaacattgcttacatgatcatttccaggcaaggagatcctaacacttattgacttggaagatagtaggatgccaagcagtgcagaaccctactggacggacagaagctgccattctgaacatttactgtgtaaggccacataagctgcagttgtataacatcataattttgttgtaaattaaaatatggcttgtataaaagggcattgaaaccttgtgtgtgtattaaaaaaacattctaagaagcaacctgtgaagacagcagctgagaaagcacaggagagaatggagaaggagtgtaatcccagcactttgggaggcctatcatgataggcaagggaagacgaaagagacagaagtgggatttttttttttttttttttttttgagatggagccttgctttgtcacccagcctagagggcagtggcatgatctcagctcactgcaacctccgcctcctgggttcaagcaattctcctgcctcagcctccctagtagctggaactacacgtgcactccacacctcgctaatttttttgtattttagcagagacaaggtttcaccgtgttgcccaggctagtctcgaactcctgagctcaggcgatccacccgcctcagcctcccaaagtgtgggataacaggcatgagccacagcgcccggcccagaaatgggatttttaaggtgtctgggaaatgtatcatattttcaccttagaaaggcttagaaagagtaccagactagaggtcagaaaacctgattccaggctggggcgttgccgctcactggttaagcaactagggccaacagcaatccccacgttaggcgagcacttggcagagtttataagattttctgggcaagtttccgctctctagggtcccattccctctctgttctggatctccctaaaagatcttcacttattgagagtggtcagaccaggcttcatagcaacagaaaggacttaaataagcagagaaagtagaggtcataattctaattcagtttcttggctaaatggagaatctgaagaatcttttggagatctggccagtagtgctaaggctctgtaatgagaggccggagcacacacagggcaggtaggtttcatgggtgtttcaagagtggagtctgacgtcacggtttgtctgggtggaacatgcatgtacttgcagagatatgttcccgtatagtgtaattgtaggtgtattaattcaggtgtcacccctctctacacggctttcctcttccattttgctaccctaggtagaagctgggtgcggtgctgagcaagtagctacaatgattggtgctgctttatagctccctggcatcccctgaatcagttaacatcccagctttcctgatagccccaccccatcacattcttatccctctcctctccaagaaagaagccagaagcctggcagtagaggaattcccagcaggctggtgtgcctagaaaggtagtttctttctttcccttccacaggcacaaaggaggccaacaaacacgcagtttcagactattctgacccttaagaaaaaagtttaagagttcaccaaactattgtgaatgagtttgattctaatcatttgctggcagggaatatggaataaaatagctcatttgcagttgtttatttcctgttgtggcttctattttcatcttttagtcgctttggtgatagtaatcaaaccctaatcatggtgccgccacaagtcacagagaccaaaataacttgcagcagagttatgacaaacaaggatggaatcagctaaagacctggctacttaatcaccggccactgccgcccagaggactgtggggctgcctcttgaccggctgctggctaggaatctagaggagagaggaagtcgagggaagttgctccaaggcccatgttttctgagcagccagggaaggcagtagagtgcacaggaagtgaccgaaaaagcaggtgaattctccacacctgccaaggggagaggcaggcttctggaggggcctgacttgagagagaaagaggaggggaaaaaaatctccaaaactcttgacacctcaaaacaatgataagtaaaagctgaaaagtgcctgtctagagaagacaggattctgcctttcagttctttgctcattgtcagtggattccagaagagaagggcagagagaggccccaaagcatgtatggatgtgtgttgatgggagtgaggacaggggtaaagatttttttcttgcacaagccaaaagaagaaaccattgaggagaccaaaaaagtactggaaaacatcaacatttcttgcacaatcatcccctgaaaaatgtgtgagtgagccctaaaccatgcacaactggcaacaatacaaatggaagtgatggcttatgaaaagaagacagtacaaggaaggctgatgggacaatcaacgcttcttggcttctcttggaagaacaggaacataagtgaatgaaaatgcatctaattcactatcaaacaaaaatactataagcccggactccacaaatattcttggattacagacaagctgtcagctgatccccaacatttgccaggtgcctatccagagcatgcaactaggtatcagggattggaatgggggcaggatgaaatgaatgttgctatggaggagatgagaaacatccagaaaaggtaaagagtgaggacaatagagacattcaaatctacagtcacatttagatgccgtttcctccaaggagggcccctggacagctgaagaacagaactgggaggggaattttactctgtataattttgtaccttttgaattgtgaaccgtgtgaatgtgttacttattcaaaaataaacagatttaaattgttttcaaatctctgcttgcttttctcatttcctgaaattcgttgttctgatgtccttgtagaaaaggacaagttggcaaggtcccacgtggaaatgatgctatagacagcttctctctctgtgaggcagttgctacaggaagaggctggtaacaacagaggccaatgtctcatcccagacagcaagggtggaggctgcttcgtcatgagcctggccagagtcagcgaggaaacatgcccatcctaatcaaaagtcattccagatatcagtcaggtgcaagtcctaacctgggatggacagcctaataaatactgctgtcagggccgggcgcagtggctcacgcctgtaatcccaggactttgggaggccaaggcgggcagatcacttgaggtcaggagtttgagaccagcctggccaacatggtgaaactccatttctactaaaaatacaaaaaaattagccaggcgtggtggcatgctcctgtaatcccagctacttgggaggctgaggcaggagaatcacttgaacccaggaggccgagggtgcagtgagctgagatcaccacactgcactctagcctgggcgacagagtgagactccatctcaaaaaaaaaaagataaatacggctgtcaggatgacacaggcacaggaaggagcctgcccaatctgagaaaatgagagctttgctttttggaacagaaacgtgttcacatgattttcaattcatttagccagcactgattcagagctgattggagtcaggatccaggagagacctctgagggttataaatgtgaggattaatcagcctttgccctcaagaagtccacagtctaggagagccacaaactctcatgaaatgggatcagtgttaccccagcagcaagaatggaggcactggctctaagaacagaaagtcaagggactcattctgtctgggagaggcctcaaaaggtttcccaaaggaagaaatattttagactagattagctgagttgactagccaggcaaaggtgatcagagtcctaattgtcctatcaaaaagaaaaaaaaaaaagaaaggattacaaatatgagccaccacacctggaacaatgcctggtgtgatggctcacgcctgtaatcccagcactttggacagctgaggtgggaggactgcctgagcccaggagttggagaccagcctgggcaacatagtgggaactcgtccctacaaaaaatacaaaaattatggccaagcgtggtggctcacgcctgtaatcccagcactttgggaggctgaggcaggtggatcacctgaggtcaagagttcgagaccagcctgaccaacatggtgaaaccctgtctctactaaatatacaaaaattagctgggcgtggtggctggcacctgtaattccagctactcaggaggctgaggcaggagaatcgcttgaacccgggaggcagaggttgcagtgagcccagactgcgccactgcactccagcctgggtgacagagagagattctatctcaataataataataataataataataataataatacaaaaattagctgggggtggtggtgcgtgcctgtagtcccagctactctggaggctgaggtgggaggatcacttgagaccctgaggtagaggctgcagtgagctaagactgcaccactgctctccagcctaagtgacagaaaaaaaaggaacgaaattttgttttctttgagctaacttttcaatacccaagccacacttatcacttaagtgtataactttataaacactcccaagccataggaagtcagtgatgaaagtgaggtccctgcagtgggtggtctgggagggcatctccctcagaaggcagttttctctgtagaaaacattggaggaaaaacactagatcgtctacggttacagagaagtttctcctcaaataactatagagatcgccacgatctccacccctcagatcaagagcaggccttacttgagtcaaactggttcatgttaggaagttgtgccagttttaagacaagtggaagggaagtaccctcagcagggaagttggctgagatgcctcagtaatgggggtacttaaataatgctctcaaatgccaacaacaaaaaattattatttgccattatcgtatagacggtgagacatacagttggctgatccctacaggtactaaaaaattgattttaaagacagcaaagcaaggaaatcagtgttgagcctaacccagatggaccctgatgggtcctggtgttatttctcactggccatgttgcagacaagttcttcattccagcttccagccactcaactgggcagctccaagttcctggtcacattgggctaccaaattatccttttctgttttctgatttttttcctatttttatctttcccattcctctgccaaaagtccttaatgggtcacttaagtgctgaattctgcctagtaagtgctggttaggatctgagctatgagacatgctggtaatcgtgattcagaacagaaagcctgcggaggggtgaatgatgttttatctgtagtagggaattgggactagagcaaaggggtcatacaggtgaccgcacatgctgcccctggcacgtgctgggacccaccgaaggagtgagggccaaggcatcttgctcattctcccaacgcagacctaggagaatagaaaggccctcagctcggctttaggattcaatagacttttctgccattgctagctataagaccttagggaagtctgtttccagtctgtctaccttcctcatacaacaaacactgaattaacaatgtcttgtgtcttctgtgtgccagactcagcgtgaggctccaagaacaaagtcctcacggtggggttgctgggaggagacgttcacaccacaagagccccagtgctatgtaaaccaagtggtatacagatgctaattatcatattatcatggattctgaggtcctagctgcccaataagcacattttgcctaatcttccgtgcctaggaaatgaatttttagaggagataattgtccaagtgatagggtaatgaagaaggaagctactttttctagtggctgggattttgtttgtgtgggggttttttgttttcagttttttgagacagagtctcgctctgtcacgcaggctggagtgctgtggcaggatcgtgactcaccgcaacctccgcctcccagattcaagcgattctcctgcctcagcctcctgagtggctgggattacagtgtgcaccaccacacttggctaatttttgtatttttagtagaaacggggtttcaccatgctggtcaagttggtctcgaacctcaagtgacctcaagtgatccgcccgcctcggtctcccaaagtgatgggattacagccatgagccaccatgcccggccccttgtgtgggttttataaggaccagttagaactctgtcaaagaggtaaggctagcgtctgagtttaaaaacaaacaaataaacctagggaaatcttttccctgttggaataagagagggataagtgaggaaacaatgtaagtgtttttagttcttttctagtactactatgagtcatacatattttcctgtgtcctggagatatctcccctggtaattatgagatacaaggaggaagtgaagagggattcattttcatggagaggagttacccagtgggcaggattctgctgtgcccaatttagttttgatccccctctatcccataaacatttcttttgaaggctttcaaagttgggggaagatgatgttatttagcattgttagagtctggtagaccataaaggaaaaatctggagaaatgcagtaaaatgaggttcaagccagaagggattataaacgttacatagcccagagagtctccatcttcagtccatcttatttggtactttttctttgctttttctattttattgatttttgaataggcaatgcatgcacaatggtacacaattccaagaatacaaaaggggaggaagaaaaagataaggcttccttctacctgggctgccagccacccatgcctctcataggcagccaccattacagccaaagaggcagaacatgaacaggcctcggctcggcgcgatggctcacgcctgtaatcccagcactttgggaggccgaggcaggagcatcacagggtcaggagatcgagaccatcctggccaacatggtgaaacgccatctctactaaaaatacaacaaattagctgggtgtggtagcacgtgcctgtagtcccagctacttgggaggctgaggcaggagaatcgcttgaacctgggaggcggaggttgcagtgagccgagatcgcgccactgcactccagcctgggtgacagagtgagactccatctcaaaaaaaaaaaaaaaaaattaggtctctgctttgctctccagtcccacttgcctggtcaatatctcaaaggcaccctgagctcattaggtcccagataggccatcttcctcctgttacaagaaagtggtcccgagccagaccacaagagagagttctttggatctcgcataagaaagaattcagggcaagtccacagtgcaaagtgaaagcaagtttattaagaaagtaaagaaatggcagggcacgatgactcacgtctgttatcccagcactttgggaggcggaggcgggcggatcaccaggtcaggagatggagaccatcctagctaacacggtgacaccctgtctctactaaaaagaaaatgaaaaactaggcgggcatggtggcacacgcctgcagtcccagctactcgggaggctgaggcaggagaatcgcttgaacctgggtggcagaggttgcagtgagctgagatcgcgccactgcactccagcctgggtgacagagcaagactccatctcaaaaaaaaaaaaaaaaaaaagtaagtaaaggaataaaagaacagctactccatagacagagcagccccaagggctgctggttgcccatttttatggttatttcttaatgacatgctaaacaaggcgtggattattcatgtgtcccctttttttagaccatatagggtaatttcctgacattacctggaatctgcaaactgtcatggcgctggtgggagtgtaacagtgaggatgaccagaggtcactcttgtcgccatcttggtggattttggccagcttctctactgcaacctgttttatcagcaaggtatttttgacctgtatcttgtgccgacctcctatctcatcctgtgacttagaatgccttaaccctctgggaatgcagccagtaggtctcagcctcattttacccagcccctattcaagatggagttgctctggttcaaactcctctaacactcccaaacaggcttttcctccagagctccacgctcagaaagctcactcctcaccatccagtgatcacaaccagaaaccaaggacaacaaacctctcccttaccccttatcctaccagccccaaagcctatccattttatctccaaaatgcctctccacttatctgcttttctccagtctcacccaccacaaccacccagcatctgtccgggactggtccacaccttagcctctgctgtcttcctcagacccacccagtccctctcccctgccaggtggtcgggctcagtgctgatttgagtcctcagacccacccagtccctctcccctgccaggcggtcgggctcagtgctgatttgagtgcacaaccacccagcggggcttctgcacgcccttggatcaaagacaaattcccttcctggccatacaaaaccctgagtgacctggagccctctccctccctcccgcgtcccctcagtactcttccttccatcccactgagcgcgttcacttacacagggtgcttaccagtcagcttcccagctgtggaatctctgccggctgcattttttgagtaaatggctgtatgtacaaaaagagttcacattcattcctctttttttcttggaatgggcagagcatgttaagtagaatttgatgatggagacgatgaagaaattccttgacgttaatctgaaattgatcacttgtttaaaattacacaaacacatcttgcttttgaaagaaccaaagggaaataccattcaatgccaaaagaggcctaggaaagcagggatgagctcatttgaaaaagccccaggagcctgatcaatgtctaggttctggctttcccagaggagcctcacttgccttgcttatgctttctgcatgcaatacctcccagtgcaaagagagggtagtcacaggctctgggtggaatgggagatccccatttgcccccacatccttcctcctcctggcacattggtctactgggtagcagccctcaggctggggggagctccccaagggttccctacccaggcctctgcctcactctccacttccagcttagttttcccctcttccgagtccctggattccaggggacaccagctctgtgagcatgaacactcagactaggggagaggccccgacagttggctgtgcgtgcccagaactgcctatccaagtagacttctgctgtcaagccagagacactaaggaacacctactcaatgagcagtaaatccctcatgacgctaggagagggtgggcacacccattccatctcccgcccaccccactccacaccccaccaatcgcactcacccttgatctcagccagctgtcccctggtgtcctccactggccttggagatgcaggagtacgggagaagcggaataaatcccaccccagcaagaaaaatacaggtcccagaggcactcaacagacatatgttcccttcctccttctctcctggtgacagtgacagataggggccccctggggcgggtggatattttcatcttccaagagaatgcactccattactccaggacttttctgtcctctccgcctccacacagccttccagcctaacactcagtctctcaaggaatattcttgacactttaaaggatctggccagcacataagccaatgtggctgcattctttaattaatatttattgagtgtccctattaggtgcctggcaagctcagagtgttgtatgtggctaaaatatc

SEQ ID NO: 6 - DNA, 13151 bp, Homo sapiens
ggcactagatggcactagaacccacacctgccacccccaggcagggctttttccttggcactggtgcagtcaccaatctcagtagctttcacgagcctacaattgaaagcacttttctctatggctttacatcttggcctttagggcagtaacccacagcctagttagttctacttcttctgccacccttcccttgtttctgttggaaagtggtgcagctattggaggatgtgcttgactgaatgtgctccctcagcttttcagtccataggatgggccccagctataccctttcactccttccctgctcaaagatcatggaagaattcctgaggtaacattttcatcttgggtgagactcattctttacaattcacccctgtggtgagctcagcctagtgcagcctctcgtttgctctgttcacacacacacacacacacacacacagtcatgcatgtatgcacatacgcacgcacacatgagaaacacaagaaagcacctttaaaaaaaattagcggatgatactttccctttgtggatggttgcacctcataccaatcatgggtttaagcttggtgaggaaagagatggacggagatagaagctggggagaaagatttgtaattatttaaacttattgaatagctatgtgcctgctccgctctgaaaatagcgcctgggttaaaagtctctgtacctcagaaggtcaccatctgtaggagaggtagatcaaaacatatcattttaatcaggaagagtttgaggtgtgggaggttacaaggcccaggcctgagatggaactagcacccacatctgacacccccggcacagggctcactcctcaaccttggagctgttgccaacctcagtaggtatgaagaatgtattgggcacacatgttgaaagcaatgtttttctagggcgtttaggagtgagagaagcaagcgcaattccctgtggtgtcccaaccacaaagcctcttctacctgtagcagacagaggaggtgacacatgagctgagtctgggatgacaagctcacaagcatttggggtcaagcattccagggagaggagtcagcctgggcaaaaccaaggcagcgctctcggtaggcctgggcctctggctagtggtttccttcaacccacacactgcgcatggaaccacagaaggcagcacagcagagcatctgccctcacgttcttcctggtggggggcctcccaaggacattctgcctcaggttcttattgtctgaggtcactgagcctcctgaaagtatttcaggaatgtggaggcctgactcactctcttccttgagttcacagtctgaagttcataaaacctcttccccctttagtcattcttattcaaataccggcccacaagtttcacagatggagctggcaggaggaatcttgggaagcatttttttgctcaggatgtgaaagtatatgaagagtttgggagatccaggagcaatcattcactaagagccagacccctgtggcaggcgctggctaaacgcagagactggctggctcgctcacagagtggagatcactggcagaagagaaatgccatgaaagcatccactctgtgcctcagtttcctcaactgtaaacagagacaataaccacaccttcttcagagaactggatggggagtgagttaatccacataaagtagttagaatacagcctgacacataataagtgctcaataaatactagtttattgttcatactattgcttattgttggcagagtgagttgtctacacactaagtggtgtggggaagaggaggcattcctggaataggactgcgtgggataaacctgaaaggaaaatgtccaatgccgtgggtgagtgtccagatggggaggcctttagacatcacacacacacagcaggaggggcagcttgggagagaagaaacccgagtggcacatctagcctgatgccaaagtatcaattcatgcacttcttccggttggaaacagttataaaaatgtccagggaattaacaaaggggatgcaggagagatatttggagtacgggatgggcatacacatagccaagcatggggtttcaaattggtgttattcaccttatttctcctgctgccgtgcaggcaatgaaattctcagtgaggcaggccacagacagatcagatgctctgttttcctcctttctgactgtagctcagtttagaggattgaaaatgctaggagacatctagcctaccctctccctgctcacaccgcaccttgcctcagagctggttttgacatctgtcctagaagacatcatccattgccttgattcatgggtatgagtctaagcaatcttaaccactgctgggattccatttggacaaggaaaagctttctctgcttttcagaacactctacagagaaaccctaactttagtaaggctctggggaccccaggggagatccagagaagtaaagcacccagcccaatggagcttccagaatgcattttgagggacagtgctttagttcttcctttgacctcagtctcttttggtcattccttgtccccattctactccaactggaaaggctgagtagctgctcctgcatatgtctgttattgcagtgacccaaagtaagaatcttaaatgaatttgaaatcccttaaaaaaagagtaaaaatagtcctagtggaaaagatggttcaggagtttcacagaagggaattagaagaagccattactgactcaaagaaaaagattactgaatagatagcagaaggtaacctctgccctactttcagaccaatgagtagatataaatgacattacactctcgcttcatgaaaagtaactggagagttgagatgaggtgattcttgaaagaaggaaaggctattagatttcttactattaatgattaaggttcctcaattttttattaaccagcctttttttctaatgacaaaatacatccttatggtacataattcaaactgtagagaagggaataaagtaagaagtaaaattccttttctccactccacaccctccttcccacacctccctgaatacttccctgcggaaaccactattaacagtttcttctccatctttctagaattgcctatgtatattccaacctcctctgacaatcctcttttttactcacccacaagaggccttccaacttggcatctcacatcatgataccgcctttgtctgggaagctcttctcctctttgcatggctccctcatggctgctacaaccttctcggaattgtcaactactcagagaggtctcctgtgacttctctatttaaacaaccccaccaccatcaccattctccaccctgacaccaccagtgtctgcccaacccttagcacaatgtccagcacacagtatttgatcaatacatgacggatgcgtgagtacattaggtacgtgcgcatgcacacatatgcatgtattctccccacaaagtataaaggggatggtattacagagataattctgtaatttgctttcctacttcacaacatataataaaaaacaataatgataatatttcttaagcacttatgttccaaggactattctaagcattttacatgtattctttcatttaattcttacaacagccccttaaggtggtactaatactacccgacttgccagataaggaaacaaagaaatggagacatggggaggttaaaacacagcttgcaagtggtagagccaatacataaatttacactaatcgtaaaatggctgtttagccttaattcacatattaaaatattttgtggcaaaatatactcaacataaaatttatctttttaataatttttaagtgtacagcttagtggcatcaagtatattcacattgttgtgcaaccatcaccaccatccatctccagaactttctcatcatcccaaactgaaactcagtacccattaaacattaactctccatgctccccttcctccagcccctggcaatcactatgttatttcctgtctctataaatttgagcactgtaggtccctcatagaagtagaataatatagtatttgtgcttttgggattggtgatgggtttgttgcacttagcaagtcttccttattaattaattaatatctaatgaataattttattgagtaaaatatttgagtgcatgatacaaaattcaaaaggcatagaataaaagagcaagttctccttctacctctgtctctaggtaccccaggggcaaccactcttcctagtgtccttccaaagatgttctatgcatgtacaattacattatttgtatgagtcatatatgtataatatatgtatagcatactatacatactgttttgtttcttgcatttcccatttaactctataccttggagatagttacatgtcaatgtacatggaactgcccctcagtaaacataatttacataatgtatccagctgtacacttatagtatattcactttgtatgtatgtttcaacagaaacataatttacagttcaaaacataaattatgtttttcttgaaatatacatacagaaagtgaacagctggatacattttcacaaactgaacatacccctataaacagtaccctgaagaagaaacattaccagcattactagtttcccaagtctctcattttttattccagacgttactcactgtcaccaatggtaactactctcctgacttaacagaatagattagttttgcgtattcctgtagttttgttgttgtggtggtttgtttgtctgtttgtttgttttttagagacaggatcttgctctgttgcccaggctgtagtggcacaatcatatctcactataacctccaactcctgggactcctgggcttaagtgatccttctgcctcggcctcccaaactgctggcattaaaggtgtgagacactgcaccaagccctgttcatgtagtttttatgaaaataatcctgctgtatacactcttatgtttggcacatttcactcatccttacacctatgagattcacccacgtcgctgaccttcagttgatccttaacaacatctttggataggtgaaggcccttgcagctgtggatgagcccagctggcatgaggtcttacatgtcatacccaccttctctcagtcttgccctcacaacctttgaatttctataaagtgctttgtaaatgccttaaagagtccacatgtatccaaaattcatctccagatgtatctaatgatgaaaaccagcagcccggagctgaggtttgtgtaaagttacatcagagtgaggaggggggaaggagcacagccttcccattctgatcagtgtctctgtggccacagctcaataagacttgctttttgaggcctcatccactcagcccagaactcaaatctcaaattccccaaacatgaggaatcatgacaaagcactggtttgcattctcttggcaaatgttactttaaaagtagagtcaaaactacttccaagtaaagagcaaagcagctttaaccaatatcagcaaagggtctaagaaaaaagatgtggctaatgtattccgtctgtttgtttgctttcttgtgccctaagactcaggagaaaatatcagtttgggaaagaagtcataacacatggggcaggaacaaaataccaacagagcgaagttgcacacgctgtccaacctggtggcctgcttatgaatttgaaatcccagaccttcacatgagtccccagcctcaccccatccctagcctggcacagacaggaatatctatttccagatatgagctgttacatagcagaaccaatctgtacatccgtgtggggccaatcgtcagtgctctgattggctcatcagccaacatgcagggctgcattcctgtggttcacccttccagaagggcctttcccaacaccacatgctgcctgtgctgtgtccagcaggagagggggaggcaaatgatgtgtctcatggcaccacaggctctgttttaccagaataatactgttctttggcccactgcatccgttctccccacatgggccttttcctcacgtggaccctaaaagaccacttctctatttacctgccaacctgtaacagataattatagtggctgccagatatcccttcaaattggtcatgatctcattcggttattctagcagcaaaaaagttacagaaaacccaagataatattaaaaaaagaaaatcatcccctggctttcacctttcttgtggcaggcaagaaaaggtaggaagaataagcataggaaaagaaaagtaagagcttgtggggcaagttgaaaacaaaccttaccaagtccagaaagaattttccatttaaatgctttataacaattttctctgatgagtagtagaatgctgaataagacatgttactttttagtgacttttcaatctggcatctattgaaaggtgttttatacccactgcagccaagaggagagggtgcaggggagatcacatactctcccagcaaggcagggatagaaagcccctgtcaccaggggctgccgtttctctggcccaggaacctgtggaggctactcctggataactacacactgttcagctgtattgcatgcaattatatcacattccttcctggaaacttctccaaaaagagagcagagatgagaaacactcatagagaaagctttcactggggcacacaagctgaactggcaggaatctgaagaaggcaaagcaatggaatgttaacctcgaatgagtgaacaggagataagaaaacatcagctgacagagcaaacaccccggaaatgtgacctgcctaccctgggaatggctagagctcttgaactagcctttaaatggaaagttcttcctgactcgggttttgaaaccaagactgagcaaaagcctcagtcttcattcctgagatgaagtttagagtgcaaaagatttcgaatgcaaaagattttgagagttggttagagcccgaggacaagcctcttgtgaacagaagttccaagagtcaacagtagctggcagcagacaacctcttcaggctgaagggtggcagaacccaagatggctagtgcagaagacatctgagagatggcccaaggctgtcctttgcttttcaaatgaggaaaaggtccagaaagggctgtctaaggtcacatagctggttaatgacagagctgggagtagagccacattgagctaagttgtattcctacatctctaccaatgtgtaacccaaatcaaaataattggggggcagaagaaaggggaaaagttatggtctttgaaagtcattagtaatcctatcattagacacataattaatatcatttgccaagatactaatgtcttaaatgtgagaggcaatgtctattgcactaatgaggtgactggtaccatggccatttatggcagatatattttttcaaatttaagactttagcatacacatatacatatggagagagaaagagagagttgatttacatatatatttcccatctaaacacacaccttgaccattttgccaggaaaataaccaaacaacttccattgaggtatacaaagaatgatgacaaagttacgtggcttatagtttaaaaagaaagtttaggctgtgtgcggtggctcaggcctgtaatcccagcactttgggaagccaaggtgggtggatcacctgaggttgggagtgtgagaccagcctgaccaacatggagaaaccctgtctctactaaaaatacaaaattagctgggcgtggtggcacatgcctgtaatcccagctgctcgggagactgaggcaggagaatcacttgaacccagaaggcagaggttgcagtgagctgagatcgcaccactgcactccagcttgggcaacaagagcaaaacacagtctcaaaaaaaaaaaaaaaaaaaaaaaagaaagacagtttaaaaacaaaattgcttgggtccctccaccttgccttttcactctctattagtttttaaagagtggcttgagtcacagtgaaggtggagaaaaagcagaagcaaagacagaagcccattcaatcaggactacatatgccctcgcaggtgaggaacagttggcccaattgtgaagtctccaggctggggcaaggagggaaggcatgcccaggaaaagcatgggtgagctgggatagtttctatgcttatttctgaaggcccatcaaggaaccaagagaaactagaatgtcctgttgagggaggatgcagactttttccctcattgtttcctaatgtaggttagaacactgatggtctagaacactgaaaaagatcttttgtattctattcaagatagatgaatgacagtacagtcacagccagttagagctagaaggacctcataagtcacctagtctgacatcttcattttccagatcaaaaaatggggtgcagatagatctagcaacttgattaaggtggccacaagctctcagagtgtgttttgccaacctctagtgggtatattggggctggggggtggggtgcacagacagcaagcactccaacaggtctgtagatctttcaaaatgcaagccaaaatgcacaaaggtgtgtgcagagtacctccctggttggtttcataaattaacttgaaaattaaattgttacaattataataattatccagtcttccaaaagtattcatctggagtgtaagcactttaaacatgatcttctgttctcctaaaggtgctggagcatgggaaggctagcccgctgccagccacatggagtgggaggatcacggagcctgaagctgagaggccacagcactgcacctgacatatattaccaacttgccatgcaacttcatctcattgactccgcattcccattttttggagtggatcacctgcagttcccttgacaactgagtgtctgtatttttctgtatcgtccagtgtgatgacaactgtctacacaaccaagtctggccagcactgaacacactcagcttccccacagtgctccaagtctcaaagcccaaactgcagccaaatcttggcagtgttgtcctctggtcaggccagagcacctttctgaaggacctttctgaacatttttagaccattcgatgaatgaccctaaattcttggcgcataattgggactgctgccatcacgccagaaacatttattaagcacttactgtgtacagtgctcaagacctgccatcttgtttccatcttgacaacaatgatgcacagtaggggttgtcattccccgtttcagagaagagtaaagctcagcagtggcccagtaacttgcccaaggccacacagctactgggtggcagaactgaattaaaccctccactttttgactctaacacctttgcctccctccttagggcgcaggcacacccagccaggctgagaggcactcaggcactctcgaacttcatgtttgtcatgcatacatatgacttccttcgacttctctgcaaatttccaccatatgcatttccatagcaacattgcaacacaaacacggtgtaatctttgtccactgcagtacatagcttgaaaggtttttttgttttgttttgttgttttgttttaaataaaaaggagctgcatatgtttacagctgacctagatcccatggcaacaaataacagatataaacttgggttcttttcctttcctttcctttctctaaatctttttattcttttctcttgtatggtaatagtttagaacatcaaaaactgggttgcaccatttgcgattaagcagggcccctattcggtgaccgctgcgccgccagcctggcgcgggcctcctgcaagacaatggccacgacctgacgcgcgagcgccagccccagcccgggagtcacgccgctggcgcttgacgcacgcggagacccgggggccgtgccccagctttgtggaacctgagggcggctcgggtcaggtcggtccccgcgggaggacaggcgcgacccgtccctcaggaccgacggcgtgtggctgcgggggcatggggtgcccctctcggcccggtcgctccagcgaggggacgctggtaagtcccacccctgccatcgccgcgggcctcctgggcacgcccggccgcgggccccagattaccctcccggcgaccctccaggcggtattgctgtcagacacattttacaaatgcaaccctccagcctaacgaaggccagcacctggcccacgcccacaggctgggaagggagagtgcagggattagaatccagcactttttaaagattttgtttcactctacttcccgtggctcctcgccccaagggcactgtggaactatctctgcccaggatcacttatctgaagccggtgttatgcttccttcccgggcagtccctgggtgcagcttccggacgggctagcttgggaggcattcctttccctggctgatgcaggaaggtgggtttgtctgtctgtggtccctggttctcccctctgattctccctcttcccagagccccagcttttaaaggcttcatattcctgacaaatggagatccactgacatgaagaaattctcaagcaactaggcaactgggattgtgcaggggcttgcccctgatcctatagtaaaaggtccagccctcactagctgaaggtgaggaggaatttcattggggaaatgtcattctttgtttcactgtcatgaatccagtgaaacttattatcaccagaaatgccccttggctgcttcctcgctgaaattgtgctgaggtatctgatggcccactgaggtagtggataggaggttggacagccaagtggtgataagaaaacctaccatttcggtagtactcactcggtgccaggtgctctgagcagctctctataacactgcctcctcacaaaccccaaaggcaggattattatactattatatagtcataatattaatatgaatatgatactattaataataaatttattcttgcttaccacgtgagggatccaaagcttgaagaggtcacctatcctgtctagatcccacttccgactctagagcctgtccaggagtgatttccccatagaagggaaagggggctgctcagcagagaaacagaaataagattgtgccaggagagatcgcattattcctcagactcaaaggccgatttgcacacctttacgataggtagagggagaagagtggaaacacccctatctctttgtccaaacccacagcgagatccaaggctcagtcaggaaggctcttcatttagtcaattgttttctgttttcagaactaaagtggaaatgacccagtgaggaaggaaaataagcacagaataagcatgatctgccttggtcacacaattaaaatacataacgctgctaaaggtacaccactcttccacccaccccttcagagtgagaaaggccctttttgccctggaagcctactgaagcattctactggggaagtattctactgaaatattctagtggggaagtccctgccgcttctgaaggaacactgaaagaaaccttattccttagagtacagtcacccagagggtttattctagaaatgcagagaggcattagagatggtatgtgaacaaaagcagggcagaggatgcacgcccagatgctgtcttggccaggttgcaattcgaatgatctaatgttttctggcttcttattgctttgcttttccaatttggtttggatatttgcattactgtattattttccctgtacaattgctgttgtctgtacacaattaggtcattttcacagttgggtgaggacacacttcagaagtgagatgagctacagctgctagctggctctctcctgggatgtgtacttagatccctttcttgttggtcccaaagactacctgtacccaggacctgaaaattttaatctaagtcatctaatgagtggaaagaactacagcatccccttgtaatggtaggtaagagatatcttgtaagttttgggttgatttgctgatcaatggttccttgggcctaaccccatattgttaagctccaaacaaaagaaaggactgtttcccagttgcttgtggcttcttggtccatgaagttctgctgaaatggaccctgggcaaggaaaaaaaaagggaagttatagagcggaggaagcgtaagctgcccctagacgtgagcccagaattttacaagcaagtatagaagctggcctttgaacaaggaccttgaagagtgagaaaaaagggatcccaaaggaatggaggcttattgtgcagatgaatactgattatggccatgttcacaaagtacactgcaacacctcaacagtgtaaaatctcactaatacataccccactaattcagccttctcaactctctggaatatgtggccttttgggtaaagccagggctaaaattcacttttgtgctatctccaaaaatgaagttgggctaaacaaatagaaaggacaggctgctattaaagtcactggggaagcccgtgactctttaagttcataatcagacatgatagtatccacctcattaaatgccccattatgggcaggaccatctctctggctcagcttgtttcctatttgcttcctctcgtggtaccttaggtctgcatctatgacattgaccttgtttctcctctcctcttttctctctctctctttttttttttttttttttttttgagacagagtcttgctcagtcacccaggctggagtgcagtggcgctatctcagctcactgcaagatccgcctcccaggttcacaccattctcctgcctcagcctcccgagtagctgggactacaggcacctgccaccacacccggctaattttttttgtatttttagtagagacagggtttcaccatgttagccagtatggtcttgatctcctgacctcgtgatctacccgcctcagcctcccaaagtgctgggattacaggcgtgagacaccacgcccggctcttttctctttttatctaaattattcattcatcatttatgcaatagatattgtgctccttctataactcaagcatgtgctaaatgctggagttacaacaagtaaatacggaacgtttgctctcagggaggtcatagtctaatg

SEQ ID NO: 7 - DNA, 12693 bp, Homo sapiens
cctttttaggcctgatctcaaatatataattggcatagatagtcttagcttctggcagaacccttacattagcaacttgacttgtagagtctggtaggaaaagtcaagtggaagtccttgaaactacaccctttcctccacttcaaggcagtagatcagaagcaaaatcacctctcagaaagtattgcaggggttagaacccctatcatgacttaaatgatgcagggtatggtagatcccattacatttcaattaattagcttgtataggcccctgcgaaagccaaatctattatcagatgatagtggatttccaaaaatcagatgatagtggatttccataaacttggccagatggtagcatccattgcagctgccatgccaaatacggtatctttactggaatataccaacatagcctttggtgtgtgggatgcagagtgacctggcaaagtggaatcacaaggaagataaaaaccagttcacttttacatggcagatacagtagtatatattcactgttttgccccaggagtatcataacagctctttgttataatatagtccataaggaccttgtcattccaacatgccatggactatcctgctggtcccttatactggtgacatcatgctgactgaagatagtgagcaggaagggacaattgccttagatactctgttaagatgcatgaataggtcagaagctgagagataagctccatcacctgtctcatcctgggttattcagatagtagcatctgaggctaagtcttgtgtgcctctatggcattagggagtgtgatcttagagagcagaagtgaaaaggaaagggaggcgaggtaggaggaagagcccaataagaggcaatagacatgacggactgctctgcaagcattgtgtgaccatcttctgagatgccttataaattactttcttggcacagtgcatctggaagaggaagggagaaaaatacatctactggcttccattggctgaaattttgccccacagggtgttatttgcactgtacttccaggttgctcattgcaggcactaaggatagtgctgaggatgtcatgccttagcatcaacagggaagccctggggtggaagtgaaaggtgatcaatgtggacatgaggccaggggctgtgagttgtatctgcctgaagttggtgagagtccaggtagagttggtctccacaaaggggactgctgttagaacaagtggccagagaccctggagacgggtgagactaaaagaatttcaagcagctatcttaatttggattcccgcagcaaaagactcagaggcaaggattccactgccagcagttcacttggtcagttttcttaagaagcactggaaggggagtggggaaatgaggtggccaataaagagtgagtgcacaatacccctgtgggaaaccggagctcagtcctgtggaaactctggatagaagtatagaatgtgtgcctgcctaggtgttcccaccagctgggtaagggggctgagattctcatccaccagctcctgaccatcactgattgagagctgcttggggaaggggttgctccattaatttcccaacacttctggtcttctgtgcttgtgggcagagcaggctccaggggccagagaaagcgctcaggtgaagggatgcaggtgctggcagttggaagacagccaccctgcacataaatgatcaagatggaggggatctggacaggatgttgcagtggcacataaaaggtgtctgatacattctccctcctttttcttttcctcttggattgtcagattttcaaatccatcattttctcttatgttgaaccaatgactcttgtctcagcctgtggcccctctttgcatatccaaacacatcaagatgctcagcagaacaaatgagtcctccttggaaggtagttgtgggcttaaacagtcattattttctcttggttatcccaaaggcagctatctctttagttattctagtaaattctattctagttagctagttaaatctattgcactttttctgcacattaaatcagatgatatgcaagctctaactacctcctgtagacgttctcatcacaactccacaagggaggcattgtacccatgtagtgaataaactgaggtctagaatgacatgcactatattcttggtaacttcttcagaaaccaaagttttagatgatttccacagatttttgtgccccttccagctgcttgagacagtatggagaatgcttttggatattgagttatcagggacattgggtagattatgggaaaatggaacagcctattaatttagtccagttctgtaagagttgggacataagatccccagtcttcacacatcccaatctcacagattacactgaacggtggtaaacaatttagatcagcttgggtatgacacgaagcttcctcttggctatttctacaacttaacattgaatggaaggaaatcacttaagccctaaaaacactgtctggcaggaggtaaaatgtcttgcttggcttcctgccccatccctcccacacccacagctgggaccatttggcccccacttcagctcccaggcctgagaccctccctgttcttcatctgcctgagttcagggacaagctgcaaactgagagcccttcttgaatatgaacatggtctggcttcccaggagaaataggtgcaaaatcaacaaccttaacacgagtctatttccagtcatttgtagatgagaagtgtgctttgggaaacttcatttttagattccagtgaattgggtatcatcagttacagagaaccaacaaaatatgaaatgtgcacataggacttccctgcaagagtagaaaggaatctgttgccttatgcatatgtatcttggactgataaattggatcacaatcaagtcttcacccttcatgttatatatgtaactgaggaggccaggtttgtttcataatggcaccttcatttttatttttttcaatgtacacactttatttgtatattaaacaagtagaaatatgtttttccccatctttctttaaacatgttcttctccccatatatcttctgtttacccatttttaacaggaacatgagcattcaacctattccattttttcttatatgcaaaggcagagtgcaactgtgataggggcaattgattcttagctttggttttggggacaatatggggtggtgggaactacggcaaactggacagtactgccttagctgaaggcagcagcccctattcaatgccaatcaattgttggcacagagaatgcaggccttatgtcgccaggttttccaaaatttcaaaaagaatccagaagtctcaattttactgtgcaattctctaattatcaaatattgctagccaatttaatttggaggttgacacccagcagaccagataaaacatatctatgggcaaaattgaaggctgggcatggtggcttatgcctttaatcccagcactttagaaggctgagatgggtggatcaacttgaggtcaggagtttgagaccagcctggccaacatggtgaaaccccgtctctactaaaaatacaaaaattagccgagtgtggtgatgggcgcctatagtcccagctacttggaaggctgaagaggagaatcacttgaacccgggaggcggaagttgcagtgagccaccattgcactccatcctgggtgacagagcggcactccatcctgggtgacagagcgacactccatctcaaacaaaaacaaaaaccaaaatcaaaaatgaaacaaaattgagcctatggctgccagttcacaatctctggttttaaaactgtcaaacagaaccctagatctactatgtagccataactgatgtggtttttctaagcagtatagaaatatagttctaagaaagtcaattatattcctagttaatgtggtactttacaaacaatagagaaatatagaattatgaaagcaaattccctatggttagtgaatcaaaataaaataaggttaggcccatcacagagtggctgcaagtgggagagaatttacattcacagggaatgtgaacagattaggaaagaggcctcaagtggacaattttgtcgggatgcagttcgccttatgtgttagctccacatgaggccaacctggttctcgagctgctttggctactggagcctcaatcccttaagaggttgatctagggtcccccctctgtcttgccagttgtccccctccacaggccgcagccccgatgagaatatccacaacctctaataatagaagccaaaatccaatggacagagagcactgtggtgtaccagtaggtggtcccatcaagggactcacagccaccattcaattcaaggtagttgtgtccattatccaggtggagaaataaaaaatcagaccaagggcaagatttgcccaacttcaccctgcagccagggccagcattggactggaacccagactcctgatctccaggccaaccatccctcctctgagccctcaccgcccaggctggcatgaaccctttcatatccgagtgctctgtgtctccactgcgattttgctcttgagggtggagagtgagtctaatcttcttgcttactggcaggcagcatggctgagtggggaggagcatgggtgttgcatctgccattcattagccttggaatgttttgaacctcagctttcttatctatgaaatggggatcatgacagtatcacctttccatggctgttgtgggtattaaatgagataacacagctaaagcatttagcagagggcttgggacataatccacaccaagtaagcattagttgcttatatccattcccatgccatctcctctgcaaggctaactcacttggcaagaggtgacccatcctctagagtggaactgaatcaaacacaggaactgaccacagagccacggcccactgtggctacttggtgcttcaggaagagaggtttctagtgtttacctggcttcagagctgtccaggtctcagccaacttcagcggtgcctcttctcactccaagatctcacactatgtgccgggtggtaatcttaataaaaagcgaccattgagggtttacccagtgccctgcgataagctctgcacagatgggttagtctgccctgaaccgcctcactcccactgagggctttcggaggcagagcctggttcatgacccccacatctcatcacagggcctggtgtgatgcctcacccaagactgtgctccttcattcatccagcgtttattggcatctcctactacctgagctgttttaggcagggaacaaagcacagataagccctcctggagcttacattctgatgaagggggcaggcaaggtatacatagggaggaaagccctggaatccagtacattaaaaacttttattaggattatctctgctgcatttagttgtatgtatcccttatggcccccaggcaggtccactcctgggcattcaagtcggtccatgtgtcaggcgtgcagggtgggtcacagcatctaggagctcagtgcagcttgggactttgggacatacgctccacctctctgagcctcagtctccttgtccatcatataaggaaatcactgattccagccttcctgggctgtggagaggattccctcagcggctgtgaaagagtgctttcttgcgggtcagccccgacaggacagacttaagggcgggagggagcccatcccgcttgccccaacgaacgcgggcgcggggctttcctcgcaggttacataaggcagccgcgggtggaggcagcagaggcgagcgcacgtccgtcgagggggaaaggggcgtggggaggcggccggggcggccggtatcccccgggcgtgagtgcgcagcgcgcgggggagcgcagggcgcggcggagtcgggtttcagagcgcgggtgactcggggcgcgggccgggagccgggattctgcccgccgccgccgctgccgagcgccgcctttgttccctgcaggaagggcgagcgcggcggccagcgctcagcgacccttcgtcctccgctaagctccaacgctctgctcgactagccgcgcgccttccggggctccgcagacccgcgagatggcaccaaggtaagacccgcttctctgcttcctcgcgtcccgggcccctccaatactcttgcccgcctcaccttttctccctcgggcacatcttgcaggaggaacaacgggcagtgctggtgtctgctgatgctgctctcggtctccacgcccctccctgctgtcacccagacccgcggtgcgacaggtaagcaacccggtcggagggtggcaccggctgcctccgcgcccgtgggggaagtcggttttggcggcggacgcggctgcgatgcgtgcctcattcctggacataaaagggagtcttgccactcagtgcgcactggcggtcccgcgggcggctacctcctggcagtgcaggggttatagctgtgaatgggatccctgggcagctggggcggttggagcgttgtctgggcacccgagatgtctgagctgggtgcggagcctccaatcttaggcagagagggacttcagaaacagcgccagcgccagcgccaacagcctcagcgcacccagcgccagcagcttaggttgtgcgtgctggctggcttctggtaagggcaggtctggtgcctctccgcacacaggtgcgaagcatgaacaccgggagggacatctggggcttttgctgctcaagaaataacggaactgaattgctcggttgcttaacccagctctgagttacctaagcggtcacgtctatcatgggcagtggctccaccggtggtggaaagagctgtggcctggaagccagagatctgatcccttccgttccccgggcctcagtttctccagcagaactcaggcggttggctgaatagtaagatataagttaaagtagacctaagttaaaatgggcctcggttaaggtcagactgcctgggtttgaactgtggctggctgagtgatcttgggcaatggatttcatcgctctgtgcctcagtttccccatctgaaaaaggcgattaattagaccattttaccttcctagaaatgttgtgaatattagagaaattagaaataatgtgcttcccatgattccagtatatactaggcacaaaataagtgatagaaattactgcttgattcttgcagtaactatgtgttggaaagcaatgcaagtatttttatttttattttagattcagggagtggtcatgtgtggttttttacaagggtatattgcacggtgctgaggtttgggcttctattaatcccatcgcaatgcaggtatttttataacattgaggttgagagaagcttagaaagtggccagtccaaaagccaggacttgaatccaggtctgtaggctcttgcccttgctcagctctttctccatgcagttttgcagaagagccatgctttctatagcttctgaccccctcccctttgaatttgggggattagtacacatcttcaattgaataagggaacagaaagtctaggaaacaacctctagtcggcccaaaggaaacgggattgagaaggtggccttggttaactctttgtttgcctgaagaagcccaagacagcccattgtctcctgggcaacaagacccaaatccgatgatagcttttcctgccagagtgtccagcctggcatttattgcagatcaaagggcagctggagtatagttttagcttctcagccccatggctcatgtcagaaagttgcaattttgcatatgatatagggccctgccaactcagtggcagaggccaactttgggttccatggtcttttgtgaactttgctgcaacttccagtttcccaaaaggaagatggatctggggataggaactttggtgtttctttctcctcctgtgtgtgtctctgggatccctcagtgtcagggctgttgtttctaacacaaaggaagccctattcccatttataatgtaaaaagggagggccagcaaaccttcaggagctgagaacggtctaaggagggccatttgcaactgatgggttttcagtgcccctttggggatgtgaaacgattcctaaaaatgtaaactatcctcctgcaaactgcatttgtaatgcaatttaatatccctaatacttataaaacactttgtatatccaggtggaggtgtgaacatgttcatatttcattcatccaatccttacaaccactccaggaggtgaggactgagaacagttactatctctgtttttcagatgaagaaacagaggtccaaagtcacaagacttctaagtggctggggtgggatttgaaccagacagtctgactccagagtccttgctcttaaccatcctagtgtgtagttagaagagcttcacggatggagaaggctttaggggttccatggtctccaatgagccccacaatctgaatgtcacaattgtaacatgagtccattgcatggcattgtgcagtcttcaaagcacaatgtcaccttcaccacgtccctggaatcaccacccagcagtgctgagaagtaaattgggctctgtcttacagaggggatgtgacttcctcaaggccgcatgactgtaactgggtagatccataatagccctctcacgtctgtgaacttctgggctggtgctgttccttccataggaccactgcccaactggctataaaaaacaattgccaagacttcatagcactatgaaccagcagtgttttaagtgccctgccatgaatgagctcagtcaatcatcacaacaaccccatgtcttatccccttttacagatgaggaaactgaggcacagtcttttgcccaagggcatgtagccttcagtaatataagcacaatttgagcccagagggtctgactccagaatctgtacttgtaaccactatgctgtatgcttaagtggggtggcttctgaaagcatgtttgtaagtgggctgttatgagcggaaatacatgttcccaacgatttggcagtttcttaaaatgttaaatatatacttaccctacaatctagaacttccactcctaagtatctacttaagggaaaggaaagcatatggccacccaaaaactcatatgtatgttcatagcagcattatttataatgaccaaaactggaaataaagttaaattcaccattagctggtgaatagataaacaaatgaggtgtatccatttaatggaatactactcagcaataaaaaggaatgaagtattgatcaatgctacaacaacatggataaaccttaataccattaagctaagtaaaagaagccagacattaaaaagcaatacattgtaagagtccctatatatgagatttctgtaaaggcagaaccacagagacagaaaacagaagcagagattgactgcaaaggggcatgaggaaactttttggggagtgttctaaaactggattgtggtggtagttgtgcaactctataaatttactaaaataatctaactatacatttaaaatgggtgaattttatggaatgtaagctatgcctcaataaagctgcttcttaaataaaagaatgtattttcccagagcatctaggccccagatctggtggggcttcaaggtggggttcctagccagcctggtacagagctggcacacagctcacaacttaaaagctgctggcctcttagggcattgattctctcagaaaatgggtccagagttctgcctgcacctccaggtctctggatcgactctccctactatccctgaatgccattgtgggcccaggacagggctcctcaggtaggggtagaacacatgcatatgggttttttgcaggtagttgatctgttaaaaagtgggtctttgtaaacttcctgatatcctgcacgccctaaaacagcacaagttcaggtattggaaaacctgggttccactcactgacttcctccatgaacttagatgagttgcttttcccactctgagcctgttttcccatctacgaagtggagaggcaagagtcactcatctctgtagtcctaatttaaaatgttgggaaacaaaacaaaataatatttttctagtttgaggtttgattatttcacatagtttagttcaacaaacccattctgtgctggccctcatgctggctgggtacagaaaggatttgggcacagagctgccccaaaggggtcatagttcacaggaagaaagaaagggccacagacaactgtaatgccatttttcctgaagtcttctcatctaccatgcagaatgtcctgtgtgcagccaatcccatccttctacaccatcctgtttaaagacacacttgtcggccgggcgcggtggctcacacctgtaatcccagcactttgggaggctggggcgggcagatcattaggtcaggagattgagaccatcctagctaacacggtgaaaccctgtctctactaaaaatacaaaaaattagccaggcatggtggcgggcgcctgtagtcccagctacttgggaggctgaggcaggagaatagcttgaacctgggaggcggaggttgcagtgagccaagatcgcgccactgcactccagcctggcaacagagggagactctgtctcaaaaaaaaaaaaaaaaaaaaagagacacttgtcagtgggtgtcacccacatggcctcttgtacctccaatggtcagggttgagctggaggacaacaccaatccttccttttcctggtaaagtttcagggtcattggaatacccaatattttagaagataagggggctattgtccaggtagggatggtggtgtcacaagtaatttgctcttgctaataaagtgttgatgattgcaaattatttgcttatgtttaaactgttttattgtgaaatacaacatccattcagaaaagtgcatgctaaaggtacagtacaatcttgtatcacagagcaaacatgtaatccagatgaagatataggataatccccagaaggtctcctaaacccctttgctgtggttttattttcccttctttctctctgaggtaaccattaccttgacattaacagtcatccctttcttgctttttaaaaatagctttactatctaagtgtgtatcccaaaattctgaagttctgttttactcgattttgaactttttaaatgcagaatctattctttcatgtctgattctttcaatgaataataagtttttgagatttattcatgctgctgtatgtggctgtagttcattgccattgctgtataatagtccattgcattagcatagcatatgttacttatccattcttctccaacatttgggttgtttccattttgggctaatgtaatagtgtcgctctgaacattcttgtacatttctctcagtgcacatgtgcatgaatttctgttggttctatacctacgagtggagtgctgaatcagagtgtgcatatcccccaactgagtagacaatgccagcatgtcttctaaatggttgtacagatccacacagctaccaagaaatgagggcctccatttcttcacatcctcaccagcacttgatcttgtcactgagcttaacttcagcatttctaatgggtgcatatttgatcttactgtagccttaatttccattttcctaattattaattaccttttcatatgtttattgaccatttagatatccagacttactttttattgaggtgaaatttacattatataacagtaaccattttgaagtgcacaattcagtgtcatttagttccttcacaatattgtgcaatcaacatctctatcaagttccaaaacattttcatcaccccaaaagaaatatctatgcccattaatcaattgctccccattccctcattttctcagcttcaggcagtcactaaactactttctgcctctatggacttgcctattctagatatttcatgaaaatggaatcatacagtgtatgacctattgtgtctgacttcttccatttaacataaagttttcatggttcactcatgttgtatcatgtgtcagtacttcatgcctttttatgactgagtaatattccagtgtatgtatataccaaattttgtttttccattcatttgttgatggacatttgggttatttctaccttttgttttttgtgaatagtgctgctctgaacatttgcatacaagtattcggatgcttgacggcctgtttctacttctttgcacctaggagcagaatttctggtcatatgataattctgtgtttcaagtatgacgaacccccaaactgttttccacagtggctgcaccatgtttacatccccaccagcaatgtatgagggctttaattatgcacatcatcgccaatgcttgttttcagtttttaaaattatagccattttagtggatataaaatggcatctcattgtggtttttatttgcaattctttctttctttcttttttctttctccttccttccctccttccttccctccctcccttccctccttccttccctccctcccttccttccttccttcccttcccttccttccttcccttcccttcccttccccttccttccttccttccttccttccttccttccttccttcctccctccctccctctctctct

SEQ ID NO: 8 - DNA, 12803 bp, Homo sapiens
gaagcagattgttgaggcctgtccataaattcctcacttgaacctgtagtgactaattctctcgggagtgtgggatcaaacccaccatggctattaagaatttaatatgaagccccagtgcctggggccgtgctttctcatcagccccgaaacagggcgaagcctgcatgtcaggcggggccaagaatgcaaagtctggagtccctttcctgagaagcttcctgggacagcagccttccctctggggaaattctcaggggaccttctgaacaagaagtgtcttttttcctgcaccagtcctaatcatagacaaagtgggaagccccttggcagagagaagtctggataaacaccacctcctggcaatgtacccttgcccctaacatctcccacgtacaactgacactccacccttcatgtacaacaggctcccagtctccaaaggtctttgtgaacgcagcgtgacccacagaaaaagaagcagaggtggggggtggtggaggaggttgggggaacagatccagtctattggtgaattttaagcaatgaacatatttttgacctgagaaagtggtcagagtgcatcaaattgagagcctgggctcctgcagccagtgagggggcagaggcccaggaagagggctctgggtgacccgggacagcagtgggtgatggggcaaagctgtctcacctactgggcttggttactcatgggactgatgggactatcagagagcatgtggcttgtgaacccaggaatgccttcttgaaacagcctcccatccttcctgtgagatccctgagagagatgaagcttcagggacaatttagtgactgagtgccactccgcctgggattgtgttaggcacttaatgtgacaaataaaatacacacggttcctcccctcaagggcagtgacaggtgagaaatacggaggtcatcctattatttcagatgtgcctgaatcccaaagttgagctctttggcaaaccagagccccacaggatccccgggccgtgtttgtaatttactagacatgtaccaactgcatcccacatatctgtccgtccctcacaagtgcatctcacccatcagagagtgctcacagctctacctccgagacacatgccctgaatttcaccacttctttcagcccctcgccctacacccagtcaccactttttctttcctggatgactgttcttgtagtctcttctccaaggagcagccagagtgatttgctctaagatagtaagtcactctcctgctaaaaccctccatggacttcccatggcccttagtgggaaacgcacactccctaccatggcccctggacaagactttcgccatctgtctcctgcccacaggacgtccttcccctccactttgccccttatgcacacgccttctttccactacaagaagatgacgcacttgtttgtttccctgggtctctgaaattgttgctcctccttggaatgtttgctcccagcttcccatccttcagatttcagctcaaaagtcacttcctcgcagaggtcctccttgacaacactaaccaaacccctgcatcactcattgcccatcatattcccttacttttatgtgcagagcacttatcaataacagaaatcatcttatttctttgtgtgtatgtttactgcctgtcagtctcctcccgccatgccccttgaggttcgtgtttctcttttatttccttactactttctacttagcacccagagctcagtgcatagtagagtctccaaacatctttgtggcctcattcattgactagcacaatgctcagacatcaaatatccatgtgaaaagagcatagagattgaatccatctactcacttgtcagaggggaaaatggagattccaagagggactgggacttgcccacagccatacaattccttcatttattcatatcagctgatacatgcaggataagaaggaggtatccgtttgaagatatggggggaagagctagtgcaaagggcctgaggcacgacctttacgggaaagcaggcaggaggtgagtgtaacagagcaatccaaggaggagaggtgtgaggggaggtggccaggcaggcagaagccaggccatgcattcgcaacttggatttagttccctctaaaccaggggtgtgaatttctctgcccacttgtgtaagatgctcagacagcatgggacctgggagactagttgggcacccataagaagccaagagtgaagatcctgtggttgagcaagtcccatgggtgtgtttgccaggacatcaaaggtgctgcaggcagcggcagccgcctgtctgagctccattaccgtgtgggaactgcacaggacccacccagttagtatgagtgcagtactcgctgtgcaattacggctgctactgctggctgaccacgtgccaaatcgctgcacagttagttactcatgccacaggctttggaccaattaagtgagcaaagagggtggttaacgaggagtaaacaatccaaatgcccatgattacactgaggctttgctctaatgcatccaagccaggagatgaggatgggcagcagggaacatggggtctcctgtcctttgttttgtatggttggcccactgaaatctctttcacccagcccaccctgtcccatactctgctatcactgtctgctgattatttttttcttgtctcctcccctcgctttttttttttttggtggaggggcgtgtgtgtgccaagttctaagcactgagattacagcaaaacaaagcagcacttatggaactgacattttaaagtcaaacaatcaggtaaatcaatatgatgcatcaggtggtaatacatgctatgaagaacactgatgctgggtaagaggaatagagagctctcagggcatgggtgctaattcatatagtgagtctagagaaggcctttttgggtgagtgcagtggctcctgcctgtaatcccagaatttggggaagctgaagcaagagggtcacttgagcccaggagtttgagacctcctgggcaatatagcacgacctcatctctacaaaaaatatatgctttttaaggctgggtatggtggctcccacttgtaatcctagcactttgggagcccgaggcgggcagatcacttgaagtcaggagcccaagaccagcctagccaacatggtgaaaccacacctctactaaaaatacaaaaaaaaaaaaaaaaaaattagccacgcgtggtggcacgtacctatagtcccagctactcagggggctgaggcaggagaatcacttgaacccgggacacagaggctgcagtgagctgagatctcgccactgcactccagcgtgggtgacagagtgagactccatctaaaatatgtatatatatattatatatatatatatgttagctgggcatggtggtgcatgcctgtgtcttagctatatgggaggctgaggcaggaggattgcttgagcccaggagggtcaaggctgcagtgagctatgatcacaccattgcactgcagcctgggcaacagagtgaggccctgtctaaaaataaaaactttttttaaaataaaggtttttttgataaagtgacacttgaacagagacctctctgaaggaagtcagggagccagccatgcagtcgctggggaagggcatcgcatgcaaagggaatggccggtacaaaggccctgagatttctgtttgcaggggtagaccagtgtgactggagcagagttagcagtatcgtaggatgatttgggattatacagctacagggaaggatgagggcaggttccaagtatggagaacagcattctcgaaagcctccagcgatgacaagtgctttctgtttttcaaagtattttacctcatttgatcctcagaacaatactgtaagggtaagaaggatagatttctttttctattgactgctgaggaccgaagctctagaatgtctaacagttcagccaggatcacataggaatattccgattcagaggcagaaatctgtggtctgcactatgctttcaggtcagattagaggctcattccttttgacaccatgccattgtgagcttccaaaacaagatccgctctcaggcaagcctctgaatgggttacaaagttcaaaatggagccaagcacaagaagagttgccaagagtgatacagaacgctctgtggggagctggtgtggaaaatcagcacacccagcgcctgtagtaatttaaccaatacagcagaaaaacgtagcttgcgtgtctttcgaagaaacctttacagaaaccctgaaaagctagaatcctccctgtgtctgatcataatttaatatttctggaataaaatccttctagaatatatgtcctttagaattcctccaagaagcttcctatggagctccagataaagaggacaatctaaaagttaatatgaaagattaaattaaaaatgccatccagaaaacaagattcccctgcaagggacgcatataacagattttgcaaatgtgtggtagatcttactcctgccatcagcacctactgaattcccgatgctattgttatcgtcattttcactacttagtttctagtggccacaacatcaactgagagtgacttgatgggctgtcaccaaatttggaaggaatgtttgcaaacatttgtataaatgtaggaaacaaaatttactttgcagggctcaggtgggagtgcgtcccaaattgcgagggagtcatcttagacactggaggggctgctgaccaagagaggcctgccatagctctcaggaagctgtagaaagtgaagtacagagatagattcaaaatttaagtcccatattgcaagtcacaaagacagatgctctgaatcaccagcactgattttcgagggagctggttctgacacgggctgctctgtgcacagtccagaaatctatgacttcatcatgttaatgagactggcagtcaacgctgggaccacacctcaagtgggcttctcctggagcattagctcccacatgccaaagagcggggagcgtttccctttaggcttatgcggcagttctcaagccactcgatctcaggacccctttacactctgtctttatcaggaatcgaaactgagaagatggccgggtgcggtggctcacacctgtaatcccagcactttgggaggcggagcgggggggtgcgcagatcacctgaggtcaggagttcaagaccagcctggccaacatggcgaaaccccatctttactaaaaatacaaaattggccaagcatggtggtgcatacctgtagtcccagctactcgggaggctgagccaggagaatcgcctgaacctgggaggtagagggtgcagtgagcagagatcacgccattgcactccagcctgggcaacaagtgcgaaactccatctcgaaagaaaaaaaaaaaaaactaagaagagtgttctaaatatttacgtggtagtttacatactgggtacaattgtatactgcttgggtgacggtgcactaaaatctcagacatcatcactatacagttcatccatgtaaccaaaaacccttgttagcccaaagttattgaaataaaaataaataaacaataaataataaataaatatttatgtggtaatttatttaaaaataacaataagcccactacatgtttcacataatcatagtattttctttttctttttggagacagggtctgactctgtcacccaggctggagtgtggtggcacaatcatagctcactgcagccttgacctcctgggcctgagccatcctcccacctcagcctctcgagtggatggggctacaggtgcacaccaccacgtcctgaacaatactttcgaagtaaaaaaaatcgtaagtgtggcgttgttttacatgtttgcaaatgtcttaaacagacacctggattctcctagctgcttattatgatatcataaggatgcagcctctggaaaatgccactgagcactcgggagagcatgagagcaatacggtaaatgtgttcttggtaactatcatgaaaaatattttgacctcatggaccatgtacaagggttatgagaccgtcccgacagggatccccagaccactccatgaaaaccttagtataatggtggaagccaaattgttggggactttgggcatattgttaaacctcttcatgcctcaattttcttgcctataaaatgtagatagtaataactgtcctcataaggctcttgtgacaataaaatgacttaatatgggtaaagtgcctgacacatagtaacagctcaataaatgctggctagtattatgaaccgctcaagagccaagtccatgggttcattgttcccccaaagcagagaatggggaaggcgtgcaggaatctttcaggaataagtgcaggcacatgtgaacaactctctcagtgagaggactttcctaggacagggaaaagtcttttttttttttttttttttgcccctattaaataagctaaacagatcagagaggccatgtgactcatcaaagtcactcagcgggtcctgtgtgtagctgctgtagctgagaatggccctcccgcacctccccaccccacactaccctctgcatccaaactcatccgagcacactagggatggaggtcctggagcatcgattttgtcctgttgtggaacatacctcatgtgcagtctcaggggccaaacgaggtctacagaacgctgtagcttaagacatccaagctctctcctccctctgtcatgccatctagaacacacttctaaattgtaattacatactaacttatgtgattactcactgacttcccctccttagtcctgggaccctctcagtctttttggtttcaatggctgtcatgtcagggatgtggcagaaactctatcaatatttagatgtctgttttaggaaagaaggaagaaataaaaccatgtgttttcattgatgaaaagaaagcaagcaacagacagctgaatgttttctgtagataattaggtgtttgagatagtgcagaaaggaggagagtacggtaaaatgttaaaacagaaaatcaaccaagagttaaggtgtttgtctaccaagagtgctggttctgcttagttttagaaacaataacaacaatgataaggacaagaagggctcacggttactgacagcttaccgtgggcctggcatggcgctaagcattctgcatgtatcgtctcactgaacgctccttatctgctgtgatgttatttccattttacacagtgcttgaatgactccagaagtcccacagccagtgagtaacacagtgcatcatggaggtgggtcatccttggaaggcctggggcatggaatacaagctggagaaggtggaaggaggctgggatgagatggtggcaggttgaggtgccaggcagaagagtaggcctgagtgcaggtgctagaagttcagcgtttctggggctgggcacaggtgagcaagataaaatgctgctgatttcttaattgtggcaccagacactgactggggcaccaggcacagagctggagcacaccatattttataaaaagaaatactaaggctcagagggagaaaaggccttgcccaaggtcacccaacaagttagagcccagcccagtcttgctcccagtccagggattttggcactgcaacaagtgcccctcttctgactaacagactcacacgcttcccccatggcaggctcccctggtccctggctccctgcagagaggatggcgtgggaagggagcaaagcagcaggcttcattccaggattcccctcccagggcaggaaggagagggctgtggggcatgaccaggcctgctgtggctgactaggggttctccaccagccccccaaacccagaacaaagcaaggttaatgagagcaaattacaaaggctctgaaaatggaagggaccctttgaaggctgcaagggtgagagctggggtgggaccagcctgctgtctctgtcctcttgtgcaatgcgcttcccccgggaacaagctggcacaggacggtgctcacagaaacatccatccctgtggtcattgctggaactctggttgggcttctactctgaatttttctacattccaattgccagaaaaatgaagatttctgattgcagacagctcagcagagttccccagccattccaagacttggggcttaaaggagatttgcggggaggagctccaccacacccagaacctctggagaacagattaaggctctgagcatcgctgttgatcatctctgcattggttcacttttctctttgtggtgaggggtggatatagtaatatgcactgacatgtatgattaagttcttagtctgatactagcacagtgctaaggggctatacaccttaactctgacaataagcctatgagatgggaatcatcaaattacccctttgggtggcttagagcagtggttatcaaagtgccttcttggactagcaacatgagcatcacttggaaatgtgttagaaatgcaaattcccaggtgctattgccttagagagcataagaatctcccccaagttgcatagcagcaagtggcagcccaggactgccccaggacccacacttctgcccactagtcactgctgcctgtgtctgtgggccctgtctccctttcacaggggtgggtgagtgatcatgggctgagagaggctgaaaggaatacaaaagaacagcacattcactaccatactctttgtaattagaaaagactggggcccggcacagtggttcatgcctataatcccagcactttgggaggccaaggcaggaggatcacttgagcccaggagttcaagaccaacctaagcaacatagccagaccctatctcaataaaaattaaaaaagaaaagattggaaacagcctaaaccagccctaggctggttaaataaactatggggtgttcatgtaatgcaacaactttttacagaaaaagagtaggaaagctttttatagatactatgaaatggtctctacaatggagtattaagtagcagaaagcaaagtgtagaacactgaatataggaaactaccatttgtataaaaaaagagacaatacgtaaacaaatttgtttatatgcaaatacacacacacactgaaagacaattcaaagaattggcacacagagacttcctagagttgactgtgcagagggatgtgaggaggacctctcatatgtgccttggtaccttttgcatgagttacctactcaaatgataaatagagtacgattcaaaagaagaagaagaaagaagaagggagaggaggaccagcctgagggcttaaaaatgccagacattgggctgaattcttacatgcatcatctcctttaatctcctcaacaacccctagagttgattactattattagtcccattttgttgacatggaaacagaggcacagagaggctaagtgactttccttgagtacagagctattgagtggaagagctgggatttgaaccaacatatgtgtgactccagagcccaagctgtaaatcactgtattactttatatgtgtgagttaatttcatcctaccaactctctttgaaagaagtgatggttttcccctttataaataagaaaatagaggcccaaaggggttatgtggcttggccaaggtcacattgctgaagcatgaccaaccaggaagagaatccctagaaaggatgtacaattgctggggtctgtagctgcaagttctcactagaagagaacccttctcaataggatagaggggaaaggctgttgtcctgtgtaaaggcagggaccatcatgtcagctgattgcccagtttctggcatagcatctggtacatgctgagcacctgaaaactttggaaggaagagagggaatgaggaaaggcaatgctgaccagtggccacccctggaaggaactctgtaagtcagctaggccagatggacaaactgcagcctagagatggggaggggctaacttaaactggtcgagtaaggaggtttgtttgtttttttgtttgtttgtttttgttttttgtttttttgggacggagtctcactctgtcacccagggtggagtgcagtggcatgatcttggcttactgcaacctccacctcccggatccaagtgattctcatgcctcagcctcctgagtagctgggactacaggcacgcaccaccactcatggctcctttttttgtattttaagtagagatggcatttcaccatgttggccaggctggtctcgaattcctgacctcaggtgatctgcccatcttggcctcccaacgtactgggattataggcgtgagccactgcaccaggcccagtaaggaattctgaagagagtggacacaagggcagataatattttttaatgacctacttacaggctgggaacggtggctcacgtctgtaatcccagcactttgggaggctgaggcgggcagatcacctgaggtcgggagtttgagaccatcctgatcaacatggagaaaccccatctctactaaaaatacaaaattagctgtgtgtggtggcacatgcctgtaatcctagctactcgggaggctgaggcagaagaattgcttgaacctaggaggccgaggttgcggtgagcagagatcgcgccattgcactccagcctgggcaacacgagcgaaacttcgtctcaaaaaaaaaaaatgacctatttaccttgggaaattttcgtgatttccttctgtctccctaacagagatggaatgggacaggaactggccaattttgattggaatgagaagaaatatccatcccaaggttaaattcagtggggaggagggtctttcagcagctgttgaggtaacagggaggcagtggatataagaaggcagctgagatataaaggagaggccagtggattcgaaatcaggggatctgggttctagtctcagctctgctttgtactagctgggttatgtgagcaagtcacttcccctccctgacccttactgtcttcatctataaatagcagagttatcgtgggacacaaataagaatacagaaagcatgcataaagtatgccgggccctgtggctcatgcctgtaatctcagcactttgggaggctaaggctggcagatcacctaaggtcagaagttcgagaccagcctgaccaacatggcaaaaccccatctctactaaaaatacaaaaattagctgggcatgatggtgcgcacctgtaatcccagctactcaggaggctgaggcaggagaatcacttgaacctgggaggcggaggttgcagtgagatgagatcgtaccactgcactccagcctgggcaacaaagcgagactgtctcaaaaaccaaaccaaaacaaacaaaaaaagaaagcatgcatagagcaaatgttaatatggggagttattaaggacacacaacaacagtactggtgacaaactgcgctgaacgacttgcctgtcgcatcagccattctcttgattccaaatgtagtgcggagctgagtccatgccggtctcctccacttgttgaaggggaattaactgtctgggctccctatgaggcttttgctgaccttccttcccccagggcagcacttaccatgttccttgcttaggtgtctgcctctctcactgacagctaattgagggcagagaccatgcagtgttcctcacttaattcttaaaccaaggacacagtgggagagatggagggaaggaaggagacatggatgcatggatggataatggacagttgaatattttcagcatccagaggaaagataattctgatgctggtaagttaacacttcttagagaaaatctatttggactgagacttaaaagagtaggtaaggtttcagtagggtgagatcgagaggttagagaggaggaaggtggttgggtaggtgagaacagcctgagctcaggcacagggcaggaaagctcaaggcatcgggcagtcatgggcagtggtctggggtcgacggatcggaaagagggctgtggcccgctgccgctggaaaggcaggtttgagccaggttgtggcaggccttgaaaattgagcaaagtgtctggactcctccatcctgcaggcaacagggcgccacagaaagttttgtaagagagaagtgacctgttctgccctgtgctcgctggcggcgtgtggaagggcgggcaccgggccaaggccagctcggggaggaggtctcaccacttgctgctctctgccgggctctcctgaagagctgctcaggatcagggcgagatgtgggaggctgtggatcctcctgcagggaaggcttccccttcagaaatggctggattggacagcaagccttccaggcctgcctgctgggcatagacccatgaggccagacttaccctccgcattccccagagcaccctcagcagcactgccccagttgccaggaagtgccttagctctgggttaaagtcccggctcttccacggaccctggggtttggactagtccctgtgcctctctcgcagcccctgtgtttcacaacttcaggaagtcccattcacacgggagacaatgaaacaatgtgcccagacttgtgcaacccagcggtcctgcttctaatagcaatttccttggctgtaccgaaaggaggacgaaggttggtgtggatcacctctgcaggccactccaagtctcaatttatagcagtctgagcaaaatgatgggctttggtaggaggtagggggccagggcctttgt

SEQ ID NO: 9 - DNA, 15 bp, Homo sapiens
aacacgtctatacgc

SEQ ID NO: 10 - DNA, 15 bp, Mus musculus
aggtgtgcgatagag

SEQ ID NO: 11 - DNA, 16 bp, Mus musculus
cgcaagtgccaagagt

SEQ ID NO: 12 - DNA, 16 bp, Homo sapiens
caagaagctggagttg

SEQ ID NO: 13 - DNA, 20 bp, Homo sapiens
gtcgactctgctatactcca

SEQ ID NO: 14 - DNA, 15 bp, Homo sapiens
aggtgtgcgatagag